European Patent Application EP 4 527 406 A1, published March 26, 2025. Title: CANCER VACCINE, TCR/CAR-T CELL THERAPY, COMPANION DIAGNOSTICS, AND CANCER ONSET RISK DIAGNOSIS BY DETECTING CIRCULATING CANCER CELLS IN BLOOD, USING A COMMON CANCER ANTIGEN COCKTAIL. Applicant: NATIONAL CANCER CENTER. Application JP. The sequence listing filed with the application follows.

SEQUENCE LISTING (224 sequences)

SEQ ID NO: 1 - protein, 9 aa, synthetic construct
FLAELAYDL

SEQ ID NO: 2 - protein, 9 aa, synthetic construct
ELFDSLFPV

SEQ ID NO: 3 - protein, 9 aa, synthetic construct
TIHDSIQYV

SEQ ID NO: 4 - protein, 9 aa, synthetic construct
VLLGLFSTI

SEQ ID NO: 5 - protein, 10 aa, synthetic construct
RIYDMENVLL

SEQ ID NO: 6 - protein, 9 aa, synthetic construct
FLIIQNAAV

SEQ ID NO: 7 - protein, 10 aa, synthetic construct
STIHDSIQYV

SEQ ID NO: 8 - protein, 9 aa, synthetic construct
FFTDVSLYI

SEQ ID NO: 9 - protein, 9 aa, synthetic construct
FLRRGPFEL

SEQ ID NO: 10 - protein, 9 aa, synthetic construct
LLQKIEVPL

SEQ ID NO: 11 - protein, 9 aa, synthetic construct
KMKPLLPRV

SEQ ID NO: 12 - protein, 9 aa, synthetic construct
TMNDSLSKI

SEQ ID NO: 13 - protein, 9 aa, synthetic construct
RLEAGDHPV

SEQ ID NO: 14 - protein, 10 aa, synthetic construct
FLLCLAGRAL

SEQ ID NO: 15 - protein, 9 aa, synthetic construct
VLDSLVSNV

SEQ ID NO: 16 - protein, 10 aa, synthetic construct
HLIDKVISTI

SEQ ID NO: 17 - protein, 10 aa, synthetic construct
SLVSNVNIEL

SEQ ID NO: 18 - protein, 9 aa, synthetic construct
MLVAAIQSA

SEQ ID NO: 19 - protein, 9 aa, synthetic construct
YIIEAFSHA

SEQ ID NO: 20 - protein, 9 aa, synthetic construct
TVDGSTFSV

SEQ ID NO: 21 - protein, 9 aa, synthetic construct
ILMVFSIWL

SEQ ID NO: 22 - protein, 9 aa, synthetic construct
VIADRPPPV

SEQ ID NO: 23 - protein, 10 aa, synthetic construct
FIFHKDLCQA

SEQ ID NO: 24 - protein, 9 aa, synthetic construct
FIFHKDLCQ

SEQ ID NO: 25 - protein, 9 aa, synthetic construct
DFSGLLEKC

SEQ ID NO: 26 - protein, 9 aa, synthetic construct
GLDEEQHSV

SEQ ID NO: 27 - protein, 9 aa, synthetic construct
YLIGHGTKV

SEQ ID NO: 28 - protein, 9 aa, synthetic construct
RLNDGQFTV

SEQ ID NO: 29 - protein, 9 aa, synthetic construct
GQFTVIQLV

SEQ ID NO: 30 - protein, 10 aa, synthetic construct
FTYEDPNEAV

SEQ ID NO: 31 - protein, 9 aa, synthetic construct
ALFTGWAAA

SEQ ID NO: 32 - protein, 9 aa, synthetic construct
YSYAGDNIV

SEQ ID NO: 33 - protein, 9 aa, synthetic construct
LQLLGFILA

SEQ ID NO: 34 - protein, 9 aa, synthetic construct
QLLTPVPSL

SEQ ID NO: 35 - protein, 9 aa, synthetic construct
LLTPVPSLV

SEQ ID NO: 36 - protein, 9 aa, synthetic construct
KLDVGNIVL

SEQ ID NO: 37 - protein, 9 aa, synthetic construct
ILSMIHPQL

SEQ ID NO: 38 - protein, 9 aa, synthetic construct
YMLEVYGSL

SEQ ID NO: 39 - protein, 10 aa, synthetic construct
KYWREYILSL

SEQ ID NO: 40 - protein, 9 aa, synthetic construct
FFTDVSLYI

SEQ ID NO: 41 - protein, 9 aa, synthetic construct
AYYPEDLFI

SEQ ID NO: 42 - protein, 9 aa, synthetic construct
AFEFVGEFF

SEQ ID NO: 43 - protein, 9 aa, synthetic construct
HYAKIAADF

SEQ ID NO: 44 - protein, 9 aa, synthetic construct
RYLTLDQVF

SEQ ID NO: 45 - protein, 9 aa, synthetic construct
IYTWIEDHF

SEQ ID NO: 46 - protein, 10 aa, synthetic construct
SYMAMIQFAI

SEQ ID NO: 47 - protein, 10 aa, synthetic construct
MYIFPVHWQF

SEQ ID NO: 48 - protein, 9 aa, synthetic construct
YIFPVHWQF

SEQ ID NO: 49 - protein, 9 aa, synthetic construct
TFDSSCHFF

SEQ ID NO: 50 - protein, 9 aa, synthetic construct
DYIGPCKYI

SEQ ID NO: 51 - protein, 9 aa, synthetic construct
HFFATKCTL

SEQ ID NO: 52 - protein, 9 aa, synthetic construct
KYFTNCKQW

SEQ ID NO: 53 - protein, 9 aa, synthetic construct
AYLEVTDVI

SEQ ID NO: 54 - protein, 9 aa, synthetic construct
KYVCVGTNM

SEQ ID NO: 55 - protein, 9 aa, synthetic construct
YYICQTLNV

SEQ ID NO: 56 - protein, 9 aa, synthetic construct
ILPYCRPTF

SEQ ID NO: 57 - protein, 9 aa, synthetic construct
DFSGLLEKC

SEQ ID NO: 58 - protein, 10 aa, synthetic construct
ADFSGLLEKC

SEQ ID NO: 59 - protein, 9 aa, synthetic construct
AWSYGIVMW

SEQ ID NO: 60 - protein, 9 aa, synthetic construct
SYGIVMWEV

SEQ ID NO: 61 - protein, 9 aa, synthetic construct
IVMWEVMSF

SEQ ID NO: 62 - protein, 10 aa, synthetic construct
WYGNRIVQEF

SEQ ID NO: 63 - protein, 9 aa, synthetic construct
YGNRIVQEF

SEQ ID NO: 64 - protein, 10 aa, synthetic construct
EFGQALFTGW

SEQ ID NO: 65 - protein, 9 aa, synthetic construct
GWAAASLCL

SEQ ID NO: 66 - protein, 9 aa, synthetic construct
CYAELGTTI

SEQ ID NO: 67 - protein, 10 aa, synthetic construct
AYMLEVYGSL

SEQ ID NO: 68 - protein, 9 aa, synthetic construct
VMSWIIPVF

SEQ ID NO: 69 - protein, 21 aa, synthetic construct
VKNQLRFLAELAYDLDVDDAP

SEQ ID NO: 70 - protein, 20 aa, synthetic construct
LLGLFSTIHDSIQYVQKNAG

SEQ ID NO: 71 - protein, 19 aa, synthetic construct
DMENVLLGLFSTIHDSIQY

SEQ ID NO: 72 - protein, 20 aa, synthetic construct
LLGLFSTIHDSIQYVQKNAG

SEQ ID NO: 73 - protein, 18 aa, synthetic construct
EVLDSLVSNVNIELLNAL

SEQ ID NO: 74 - protein, 15 aa, synthetic construct
IILMVFSIWLYRHRK

SEQ ID NO: 75 - protein, 20 aa, synthetic construct
YLEVTDVIADRPPPVIRQGP

SEQ ID NO: 76 - protein, 15 aa, synthetic construct
LSGLDEEQHSVRTYE

SEQ ID NO: 77 - protein, 17 aa, synthetic construct
ALDSFLRLNDGQFTVIQ

SEQ ID NO: 78 - protein, 18 aa, synthetic construct
LIQEDILPYCRPTFPTSN

SEQ ID NO: 79 - protein, 15 aa, synthetic construct
SYGIVMWEVMSFGER

SEQ ID NO: 80 - protein, 17 aa, synthetic construct
VGALCYAELGTTISKSG

SEQ ID NO: 81 - protein, 580 aa, Homo sapiens
MAGTVRTACLVVAMLLSLDFPGQAQPPPPPPDATCHQVRSFFQRLQPGLKWVPETPVPGSDLQVCLPKGPTCCSRKMEEKYQLTARLNMEQLLQSASMELKFLIIQNAAVFQEAFEIVVRHAKNYTNAMFKNNYPSLTPQAFEFVGEFFTDVSLYILGSDINVDDMVNELFDSLFPVIYTQLMNPGLPDSALDINECLRGARRDLKVFGNFPKLIMTQVSKSLQVTRIFLQALNLGIEVINTTDHLKFSKDCGRMLTRMWYCSYCQGLMMVKPCGGYCNVVMQGCMAGVVEIDKYWREYILSLEELVNGMYRIYDMENVLLGLFSTIHDSIQYVQKNAGKLTTTIGKLCAHSQQRQYRSAYYPEDLFIDKKVLKVAHVEHEETLSSRRRELIQKLKSFISFYSALPGYICSHSPVAENDTLCWNGQELVERYSQKAARNGMKNQFNLHELKMKGPEPVVSQIIDKLKHINQLLRTMSMPKGRVLDKNLDEEGFESGDCGDDEDECIGGSGDGMIKVKNQLRFLAELAYDLDVDDAPGNSQQATPKDNEISTFHNLGNVHSPLKLLTSMAISVVCFFFLVH

SEQ ID NO: 82 - protein, 1615 aa, Homo sapiens
MIAEPAHFYLFGLICLCSGSRLRQEDFPPRIVEHPSDLIVSKGEPATLNCKAEGRPTPTIEWYKGGERVETDKDDPRSHRMLLPSGSLFFLRIVHGRKSRPDEGVYVCVARNYLGEAVSHNASLEVAILRDDFRQNPSDVMVAVGEPAVMECQPPRGHPEPTISWKKDGSPLDDKDERITIRGGKLMITYTRKSDAGKYVCVGTNMVGERESEVAELTVLERPSFVKRPSNLAVTVDDSAEFKCEARGDPVPTVRWRKDDGELPKSRYEIRDDHTLKIRKVTAGDMGSYTCVAENMVGKAEASATLTVQVGSEPPHFVVKPRDQVVALGRTVTFQCEATGNPQPAIFWRREGSQNLLFSYQPPQSSSRFSVSQTGDLTITNVQRSDVGYYICQTLNVAGSIITKAYLEVTDVIADRPPPVIRQGPVNQTVAVDGTFVLSCVATGSPVPTILWRKDGVLVSTQDSRIKQLENGVLQIRYAKLGDTGRYTCIASTPSGEATWSAYIEVQEFGVPVQPPRPTDPNLIPSAPSKPEVTDVSRNTVTLSWQPNLNSGATPTSYIIEAFSHASGSSWQTVAENVKTETSAIKGLKPNAIYLFLVRAANAYGISDPSQISDPVKTQDVLPTSQGVDHKQVQRELGNAVLHLHNPTVLSSSSIEVHWTVDQQSQYIQGYKILYRPSGANHGESDWLVFEVRTPAKNSVVIPDLRKGVNYEIKARPFFNEFQGADSEIKFAKTLEEAPSAPPQGVTVSKNDGNGTAILVSWQPPPEDTQNGMVQEYKVWCLGNETRYHINKTVDGSTFSVVIPFLVPGIRYSVEVAASTGAGSGVKSEPQFIQLDAHGNPVSPEDQVSLAQQISDVVKQPAFIAGIGAACWIILMVFSIWLYRHRKKRNGLTSTYAGIRKVPSFTFTPTVTYQRGGEAVSSGGRPGLLNISEPAAQPWLADTWPNTGNNHNDCSISCCTAGNGNSDSNLTTYSRPADCIANYNNQLDNKQTNLMLPESTVYGDVDLSNKINEMKTFNSPNLKDGRFVNPSGQPTPYATTQLIQSNLSNNMNNGSGDSGEKHWKPLGQQKQEVAPVQYNIVEQNKLNKDYRANDTVPPTIPYNQSYDQNTGGSYNSSDRGSSTSGSQGHKKGARTPKVPKQGGMNWADLLPPPPAHPPPHSNSEEYNISVDESYDQEMPCPVPPARMYLQQDELEEEEDERGPTPPVRGAASSPAAVSYSHQSTATLTPSPQEELQPMLQDCPEETGHMQHQPDRRRQPVSPPPPPRPISPPHTYGYISGPLVSDMDTDAPEEEEDEADMEVAKMQTRRLLLRGLEQTPASSVGDLESSVTGSMINGWGSASEEDNISSGRSSVSSSDGSFFTDADFAQAVAAAAEYAGLKVARRQMQDAAGRRHFHASQCPRPTSPVSTDSNMSAAVMQKTRPAKKLKHQPGHLRRETYTDDLPPPPVPPPAIKSPTAQSKTQLEVRPVVVPKLPSMDARTDRSSDRKGSSYKGREVLDGRQVVDMRTNPGDPREAQEQQNDGKGRGNKAAKRDLPPAKTHLIQEDILPYCRPTFPTSNNPRDPSSSSSMSSRGSGSRQREQANVGRRNIAEMQVLGGYERGEDNNEELEETES

SEQ ID NO: 83 - protein, 1651 aa, Homo sapiens
MKWKHVPFLVMISLLSLSPNHLFLAQLIPDPEDVERGNDHGTPIPTSDNDDNSLGYTGSRLRQEDFPPRIVEHPSDLIVSKGEPATLNCKAEGRPTPTIEWYKGGERVETDKDDPRSHRMLLPSGSLFFLRIVHGRKSRPDEGVYVCVARNYLGEAVSHNASLEVAILRDDFRQNPSDVMVAVGEPAVMECQPPRGHPEPTISWKKDGSPLDDKDERITIRGGKLMITYTRKSDAGKYVCVGTNMVGERESEVAELTVLERPSFVKRPSNLAVTVDDSAEFKCEARGDPVPTVRWRKDDGELPKSRYEIRDDHTLKIRKVTAGDMGSYTCVAENMVGKAEASATLTVQEPPHFVVKPRDQVVALGRTVTFQCEATGNPQPAIFWRREGSQNLLFSYQPPQSSSRFSVSQTGDLTITNVQRSDVGYYICQTLNVAGSIITKAYLEVTDVIADRPPPVIRQGPVNQTVAVDGTFVLSCVATGSPVPTILWRKDGVLVSTQDSRIKQLENGVLQIRYAKLGDTGRYTCIASTPSGEATWSAYIEVQEFGVPVQPPRPTDPNLIPSAPSKPEVTDVSRNTVTLSWQPNLNSGATPTSYIIEAFSHASGSSWQTVAENVKTETSAIKGLKPNAIYLFLVRAANAYGISDPSQISDPVKTQDVLPTSQGVDHKQVQRELGNAVLHLHNPTVLSSSSIEVHWTVDQQSQYIQGYKILYRPSGANHGESDWLVFEVRTPAKNSVVIPDLRKGVNYEIKARPFFNEFQGADSEIKFAKTLEEAPSAPPQGVTVSKNDGNGTAILVSWQPPPEDTQNGMVQEYKVWCLGNETRYHINKTVDGSTFSVVIPFLVPGIRYSVEVAASTGAGSGVKSEPQFIQLDAHGNPVSPEDQVSLAQQISDVVKQPAFIAGIGAACWIILMVFSIWLYRHRKKRNGLTSTYAGIRKVPSFTFTPTVTYQRGGEAVSSGGRPGLLNISEPAAQPWLADTWPNTGNNHNDCSISCCTAGNGNSDSNLTTYSRPADCIANYNNQLDNKQTNLMLPESTVYGDVDLSNKINEMKTFNSPNLKDGRFVNPSGQPTPYATTQLIQSNLSNNMNNGSGDSGEKHWKPLGQQKQEVAPVQYNIVEQNKLNKDYRANDTVPPTIPYNQSYDQNTGGSYNSSDRGSSTSGSQGHKKGARTPKVPKQGGMNWADLLPPPPAHPPPHSNSEEYNISVDESYDQEMPCPVPPARMYLQQDELEEEEDERGPTPPVRGAASSPAAVSYSHQSTATLTPSPQEELQPMLQDCPEETGHMQHQPDRRRQPVSPPPPPRPISPPHTYGYISGPLVSDMDTDAPEEEEDEADMEVAKMQTRRLLLRGLEQTPASSVGDLESSVTGSMINGWGSASEEDNISSGRSSVSSSDGSFFTDADFAQAVAAAAEYAGLKVARRQMQDAAGRRHFHASQCPRPTSPVSTDSNMSAAVMQKTRPAKKLKHQPGHLRRETYTDDLPPPPVPPPAIKSPTAQSKTQLEVRPVVVPKLPSMDARTDRSSDRKGSSYKGREVLDGRQVVDMRTNPGDPREAQEQQNDGKGRGNKAAKRDLPPAKTHLIQEDILPYCRPTFPTSNNPRDPSSSSSMSSRGSGSRQREQANVGRRNIAEMQVLGGYERGEDNNEELEETES

SEQ ID NO: 84 - protein, 987 aa, Homo sapiens
MELRVLLCWASLAAALEETLLNTKLETADLKWVTFPQVDGQWEELSGLDEEQHSVRTYEVCDVQRAPGQAHWLRTGWVPRRGAVHVYATLRFTMLECLSLPRAGRSCKETFTVFYYESDADTATALTPAWMENPYIKVDTVAAEHLTRKRPGAEATGKVNVKTLRLGPLSKAGFYLAFQDQGACMALLSLHLFYKKCAQLTVNLTRFPETVPRELVVPVAGSCVVDAVPAPGPSPSLYCREDGQWAEQPVTGCSCAPGFEAAEGNTKCRACAQGTFKPLSGEGSCQPCPANSHSNTIGSAVCQCRVGYFRARTDPRGAPCTTPPSAPRSVVSRLNGSSLHLEWSAPLESGGREDLTYALRCRECRPGGSCAPCGGDLTFDPGPRDLVEPWVVVRGLRPDFTYTFEVTALNGVSSLATGPVPFEPVNVTTDREVPPAVSDIRVTRSSPSSLSLAWAVPRAPSGAVLDYEVKYHEKGAEGPSSVRFLKTSENRAELRGLKRGASYLVQVRARSEAGYGPFGQEHHSQTQLDESEGWREQLALIAGTAVVGVVLVLVVIVVAVLCLRKQSNGREAEYSDKHGQYLIGHGTKVYIDPFTYEDPNEAVREFAKEIDVSYVKIEEVIGAGEFGEVCRGRLKAPGKKESCVAIKTLKGGYTERQRREFLSEASIMGQFEHPNIIRLEGVVTNSMPVMILTEFMENGALDSFLRLNDGQFTVIQLVGMLRGIASGMRYLAEMSYVHRDLAARNILVNSNLVCKVSDFGLSRFLEENSSDPTYTSSLGGKIPIRWTAPEAIAFRKFTSASDAWSYGIVMWEVMSFGERPYWDMSNQDVINAIEQDYRLPPPPDCPTSLHQLMLDCWQKDRNARPRFPQVVSALDKMIRNPASLKIVARENGGASHPLLDQRQPHYSAFGSVGEWLRAIKMGRYEESFAAAGFGSFELVSQISAEDLLRIGVTLAGHQKKILASVQHMKSQAKPGTPGGTGGPAPQY

SEQ ID NO: 85 - protein, 211 aa, Homo sapiens
MANAGLQLLGFILAFLGWIGAIVSTALPQWRIYSYAGDNIVTAQAMYEGLWMSCVSQSTGQIQCKVFDSLLNLSSTLQATRALMVVGILLGVIAIFVATVGMKCMKCLEDDEVQKMRMAVIGGAIFLLAGLAILVATAWYGNRIVQEFYDPMTPVNARYEFGQALFTGWAAASLCLLGGALLCCSCPRKTTSYPTPRPYPKPAPSSGKDYV

SEQ ID NO: 86 - protein, 507 aa, Homo sapiens
MAGAGPKRRALAAPAAEEKEEAREKMLAAKSADGSAPAGEGEGVTLQRNITLLNGVAIIVGTIIGSGIFVTPTGVLKEAGSPGLALVVWAACGVFSIVGALCYAELGTTISKSGGDYAYMLEVYGSLPAFLKLWIELLIIRPSSQYIVALVFATYLLKPLFPTCPVPEEAAKLVACLCVLLLTAVNCYSVKAATRVQDAFAAAKLLALALIILLGFVQIGKGDVSNLDPNFSFEGTKLDVGNIVLALYSGLFAYGGWNYLNFVTEEMINPYRNLPLAIIISLPIVTLVYVLTNLAYFTTLSTEQMLSSEAVAVDFGNYHLGVMSWIIPVFVGLSCFGSVNGSLFTSSRLFFVGSREGHLPSILSMIHPQLLTPVPSLVFTCVMTLLYAFSKDIFSVINFFSFFNWLCVALAIIGMIWLRHRKPELERPIKVNLALPVFFILACLFLIAVSFWKTPVECGIGFTIILSGLPVYFFGVWWKNKPKWLLQGIFSTTVLCQKLMQVVPQET

SEQ ID NO: 87 - protein, 609 aa, Homo sapiens
MKWVESIFLIFLLNFTESRTLHRNEYGIASILDSYQCTAEISLADLATIFFAQFVQEATYKEVSKMVKDALTAIEKPTGDEQSSGCLENQLPAFLEELCHEKEILEKYGHSDCCSQSEEGRHNCFLAHKKPTPASIPLFQVPEPVTSCEAYEEDRETFMNKFIYEIARRHPFLYAPTILLWAARYDKIIPSCCKAENAVECFQTKAATVTKELRESSLLNQHACAVMKNFGTRTFQAITVTKLSQKFTKVNFTEIQKLVLDVAHVHEHCCRGDVLDCLQDGEKIMSYICSQQDTLSNKITECCKLTTLERGQCIIHAENDEKPEGLSPNLNRFLGDRDFNQFSSGEKNIFLASFVHEYSRRHPQLAVSVILRVAKGYQELLEKCFQTENPLECQDKGEEELQKYIQESQALAKRSCGLFQKLGEYYLQNAFLVAYTKKAPQLTSSELMAITRKMAATAATCCQLSEDKLLACGEGAADIIIGHLCIRHEMTPVNPGVGQCCTSSYANRRPCFSSLVVDETYVPPAFSDDKFIFHKDLCQAQGVALQTMKQEFLINLVKQKPQITEEQLEAVIADFSGLLEKCCQGQEQEVCFAEEGQKLISKTRAALGV

SEQ ID NO: 88 - protein, 683 aa, Homo sapiens
MALFVRLLALALALALGPAATLAGPAKSPYQLVLQHSRLRGRQHGPNVCAVQKVIGTNRKYFTNCKQWYQRKICGKSTVISYECCPGYEKVPGEKGCPAALPLSNLYETLGVVGSTTTQLYTDRTEKLRPEMEGPGSFTIFAPSNEAWASLPAEVLDSLVSNVNIELLNALRYHMVGRRVLTDELKHGMTLTSMYQNSNIQIHHYPNGIVTVNCARLLKADHHATNGVVHLIDKVISTITNNIQQIIEIEDTFETLRAAVAASGLNTMLEGNGQYTLLAPTNEAFEKIPSETLNRILGDPEALRDLLNNHILKSAMCAEAIVAGLSVETLEGTTLEVGCSGDMLTINGKAIISNKDILATNGVIHYIDELLIPDSAKTLFELAAESDVSTAIDLFRQAGLGNHLSGSERLTLLAPLNSVFKDGTPPIDAHTRNLLRNHIIKDQLASKYLYHGQTLETLGGKKLRVFVYRNSLCIENSCIAAHDKRGRYGTLFTMDRVLTPPMGTVMDVLKGDNRFSMLVAAIQSAGLTETLNREGVYTVFAPTNEAFRALPPRERSRLLGDAKELANILKYHIGDEILVSGGIGALVRLKSLQGDKLEVSLKNNVVSVNKEPVAEPDIMATNGVVHVITNVLQPPANRPQERGDELADSALEIFKQASAFSRASQRSVRLAPVYQKLLERMKH

SEQ ID NO: 89 - protein, 303 aa, Homo sapiens
MRAWIFFLLCLAGRALAAPQQEALPDETEVVEETVAEVTEVSVGANPVQVEVGEFDDGAEETEEEVVAENPCQNHHCKHGKVCELDENNTPMCVCQDPTSCPAPIGEFEKVCSNDNKTFDSSCHFFATKCTLEGTKKGHKLHLDYIGPCKYIPPCLDSELTEFPLRMRDWLKNVLVTLYERDEDNNLLTEKQKLRVKKIHENEKRLEAGDHPVELLARDFEKNYNMYIFPVHWQFGQLDQHPIDGYLSHTELAPLRAPLIPMEHCTTRFFETCDLDNDKYIALDEWAGCFGIKQKDIDKDLVI

SEQ ID NO: 90 - protein, 763 aa, Homo sapiens
MKTSPRRPLILKRRRLPLPVQNAPSETSEEEPKRSPAQQESNQAEASKEVAESNSCKFPAGIKIINHPTMPNTQVVAIPNNANIHSIITALTAKGKESGSSGPNKFILISCGGAPTQPPGLRPQTQTSYDAKRTEVTLETLGPKPAARDVNLPRPPGALCEQKRETCADGEAAGCTINNSLSNIQWLRKMSSDGLGSRSIKQEMEEKENCHLEQRQVKVEEPSRPSASWQNSVSERPPYSYMAMIQFAINSTERKRMTLKDIYTWIEDHFPYFKHIAKPGWKNSIRHNLSLHDMFVRETSANGKVSFWTIHPSANRYLTLDQVFKPLDPGSPQLPEHLESQQKRPNPELRRNMTIKTELPLGARRKMKPLLPRVSSYLVPIQFPVNQSLVLQPSVKVPLPLAASLMSSELARHSKRVRIAPKVLLAEEGIAPLSSAGPGKEEKLLFGEGFSPLLPVQTIKEEEIQPGEEMPHLARPIKVESPPLEEWPSPAPSFKEESSHSWEDSSQSPTPRPKKSYSGLRSPTRCVSEMLVIQHRERRERSRSRRKQHLLPPCVDEPELLFSEGPSTSRWAAELPFPADSSDPASQLSYSQEVGGPFKTPIKETLPISSTPSKSVLPRTPESWRLTPPAKVGGLDFSPVQTSQGASDPLPDPLGLMDLSTTPLQSAPPLESPQRLLSSEPLDLISVPFGNSSPSDIDVPKPGSPEPQVSGLAANRSLTEGLVLDTMNDSLSKILLDISFPGLDEDPLGPDNINWSQFIPELQ

SEQ ID NO: 91 - protein, 858 aa, Homo sapiens
MSVVGLDVGSQSCYIAVARAGGIETIANEFSDRCTPSVISFGSKNRTIGVAAKNQQITHANNTVSNFKRFHGRAFNDPFIQKEKENLSYDLVPLKNGGVGIKVMYMGEEHLFSVEQITAMLLTKLKETAENSLKKPVTDCVISVPSFFTDAERRSVLDAAQIVGLNCLRLMNDMTAVALNYGIYKQDLPSLDEKPRIVVFVDMGHSAFQVSACAFNKGKLKVLGTAFDPFLGGKNFDEKLVEHFCAEFKTKYKLDAKSKIRALLRLYQECEKLKKLMSSNSTDLPLNIECFMNDKDVSGKMNRSQFEELCAELLQKIEVPLYSLLEQTHLKVEDVSAVEIVGGATRIPAVKERIAKFFGKDISTTLNADEAVARGCALQCAILSPAFKVREFSVTDAVPFPISLIWNHDSEDTEGVHEVFSRNHAAPFSKVLTFLRRGPFELEAFYSDPQGVPYPEAKIGRFVVQNVSAQKDGEKSRVKVKVRVNTHGIFTISTASMVEKVPTEENEMSSEADMECLNQRPPENPDTDKNVQQDNSEAGTQPQVQTDAQQTSQSPPSPELTSEENKIPDADKANEKKVDQPPEAKKPKIKVVNVELPIEANLVWQLGKDLLNMYIETEGKMIMQDKLEKERNDAKNAVEEYVYEFRDKLCGPYEKFICEQDHQNFLRLLTETEDWLYEEGEDQAKQAYVDKLEELMKIGTPVKVRFQEAEERPKMFEELGQRLQHYAKIAADFRNKDEKYNHIDESEMKKVEKSVNEVMEWMNNVMNAQAKKSLDQDPVVRAQEIKTKIKELNNTCEPVVTQPKPKIESPKLERTPNGPNIDKKEEDLEDKNNFGAEPPHQNGECYPNEKNSVNMDLD

SEQ ID NO: 92 - DNA, 1743 bp, Homo sapiens
  source 1..1743: mol_type = other DNA
atggccgggaccgtgcgcaccgcgtgcttggtggtggcgatgctgctcagcttggacttcccgggacaggcgcagcccccgccgccgccgccggacgccacctgtcaccaagtccgctccttcttccagagactgcagcccggactcaagtgggtgccagaaactcccgtgccaggatcagatttgcaagtatgtctccctaagggcccaacatgctgctcaagaaagatggaagaaaaataccaactaacagcacgattgaacatggaacagctgcttcagtctgcaagtatggagctcaagttcttaattattcagaatgctgcggttttccaagaggcctttgaaattgttgttcgccatgccaagaactacaccaatgccatgttcaagaacaactacccaagcctgactccacaagcttttgagtttgtgggtgaatttttcacagatgtgtctctctacatcttgggttctgacatcaatgtagatgacatggtcaatgaattgtttgacagcctgtttccagtcatctatacccagctaatgaacccaggcctgcctgattcagccttggacatcaatgagtgcctccgaggagcaagacgtgacctgaaagtatttgggaatttccccaagcttattatgacccaggtttccaagtcactgcaagtcactaggatcttccttcaggctctgaatcttggaattgaagtgatcaacacaactgatcacctgaagttcagtaaggactgtggccgaatgctcaccagaatgtggtactgctcttactgccagggactgatgatggttaaaccctgtggcggttactgcaatgtggtcatgcaaggctgtatggcaggtgtggtggagattgacaagtactggagagaatacattctgtcccttgaagaacttgtgaatggcatgtacagaatctatgacatggagaacgtactgcttggtctcttttcaacaatccatgattctatccagtatgtccagaagaatgcaggaaagctgaccaccactattggcaagttatgtgcccattctcaacaacgccaatatagatctgcttattatcctgaagatctctttattgacaagaaagtattaaaagttgctcatgtagaacatgaagaaaccttatccagccgaagaagggaactaattcagaagttgaagtctttcatcagcttctatagtgctttgcctggctacatctgcagccatagccctgtggcggaaaacgacaccctttgctggaatggacaagaactcgtggagagatacagccaaaaggcagcaaggaatggaatgaaaaaccagttcaatctccatgagctgaaaatgaagggccctgagccagtggtcagtcaaattattgacaaactgaagcacattaaccagctcctgagaaccatgtctatgcccaaaggtagagttctggataaaaacctggatgaggaagggtttgaaagtggagactgcggtgatgatgaagatgagtgcattggaggctctggtgatggaatgataaaagtgaagaatcagctccgcttccttgcagaactggcctatgatctggatgtggatgatgcgcctggaaacagtcagcaggcaactccgaaggacaacgagataagcacctttcacaacctcgggaacgttcattccccgctgaagcttctcaccagcatggccatctcggtggtgtgcttcttcttcctggtgcactga

SEQ ID NO: 93 - DNA, 4848 bp, Homo sapiens
  source 1..4848: mol_type = other DNA
atgattgcggagcccgctcacttttacctgtttggattaatatgtctctgttcaggctcccgtcttcgtcaggaagattttccacctcgcattgttgaacacccttcagacctgattgtctcaaaaggagaacctgcaactttgaactgcaaagctgaaggccgccccacacccactattgaatggtacaaagggggagagagagtggagacagacaaagatgaccctcgctcacaccgaatgttgctgccgagtggatctttatttttcttacgtatagtacatggacggaaaagtagacctgatgaaggagtctatgtctgtgtagcaaggaattaccttggagaggctgtgagccacaatgcatcgctggaagtagccatacttcgggatgacttcagacaaaacccttcggatgtcatggttgcagtaggagagcctgcagtaatggaatgccaacctccacgaggccatcctgagcccaccatttcatggaagaaagatggctctccactggatgataaagatgaaagaataactatacgaggaggaaagctcatgatcacttacacccgtaaaagtgacgctggcaaatatgtttgtgttggtaccaatatggttggggaacgtgagagtgaagtagccgagctgactgtcttagagagaccatcatttgtgaagagacccagtaacttggcagtaactgtggatgacagtgcagaatttaaatgtgaggcccgaggtgaccctgtacctacagtacgatggaggaaagatgatggagagctgcccaaatccagatatgaaatccgagatgatcataccttgaaaattaggaaggtgacagctggtgacatgggttcatacacttgtgttgcagaaaatatggtgggcaaagctgaagcatctgctactctgactgttcaagttgggtctgaacctccacattttgttgtgaaaccccgtgaccaggttgttgctttgggacggactgtaacttttcagtgtgaagcaaccggaaatcctcaaccagctattttctggaggagagaagggagtcagaatctacttttctcatatcaaccaccacagtcatccagccgattttcagtctcccagactggcgacctcacaattactaatgtccagcgatctgatgttggttattacatctgccagactttaaatgttgctggaagcatcatcacaaaggcatatttggaagttacagatgtgattgcagatcggcctcccccagttattcgacaaggtcctgtgaatcagactgtagccgtggatggcactttcgtcctcagctgtgtggccacaggcagtccagtgcccaccattctgtggagaaaggatggagtcctcgtttcaacccaagactctcgaatcaaacagttggagaatggagtactgcagatccgatatgctaagctgggtgatactggtcggtacacctgcattgcatcaacccccagtggtgaagcaacatggagtgcttacattgaagttcaagaatttggagttccagttcagcctccaagacctactgacccaaatttaatccctagtgccccatcaaaacctgaagtgacagatgtcagcagaaatacagtcacattatcgtggcaaccaaatttgaattcaggagcaactccaacatcttatattatagaagccttcagccatgcatctggtagcagctggcagaccgtagcagagaatgtgaaaacagaaacatctgccattaaaggactcaaacctaatgcaatttaccttttccttgtgagggcagctaatgcatatggaattagtgatccaagccaaatatcagatccagtgaaaacacaagatgtcctaccaacaagtcagggggtggaccacaagcaggtccagagagagctgggaaatgctgttctgcacctccacaaccccaccgtcctttcttcctcttccatcgaagtgcactggacagtagatcaacagtctcagtatatacaaggatataaaattctctatcggccatctggagccaaccacggagaatcagactggttagtttttgaagtgaggacgccagccaaaaacagtgtggtaatccctgatctcagaaagggagtcaactatgaaattaaggctcgccctttttttaatgaatttcaaggagcagatagtgaaatcaagtttgccaaaaccctggaagaagcacccagtgccccaccccaaggtgtaactgtatccaagaatgatggaaacggaactgcaattctagttagttggcagccacctccagaagacactcaaaatggaatggtccaagagtataaggtttggtgtctgggcaatgaaactcgataccacatcaacaaaacagtggatggttccaccttttccgtggtcattccctttcttgttcctggaatccgatacagtgtggaagtggcagccagcactggggctgggtctggggtaaagagtgagcctcagttcatccagctggatgcccatggaaaccctgtgtcacctgaggaccaagtcagcctcgctcagcagatttcagatgtggtgaagcagccggccttcatagcaggtattggagcagcctgttggatcatcctcatggtcttcagcatctggctttatcgacaccgcaagaagagaaacggacttactagtacctacgcgggtatcagaaaagtcccgtcttttaccttcacaccaacagtaacttaccagagaggaggcgaagctgtcagcagtggagggaggcctggacttctcaacatcagtgaacctgccgcgcagccatggctggcagacacgtggcctaatactggcaacaaccacaatgactgctctatcagctgctgcacggcaggcaatggaaacagcgacagcaacctcactacctacagtcgcccagctgattgtatagcaaattataacaaccaactggataacaaacaaacaaatctgatgctccctgagtcaactgtttatggtgatgtggaccttagtaacaaaatcaatgagatgaaaaccttcaatagcccaaatctgaaggatgggcgttttgtcaatccatcagggcagcctactccttacgccaccactcagctcatccagtcaaacctcagcaacaacatgaacaatggcagcggggactctggcgagaagcactggaaaccactgggacagcagaaacaagaagtggcaccagttcagtacaacatcgtggagcaaaacaagctgaacaaagattatcgagcaaatgacacagttcctccaactatcccatacaaccaatcatacgaccagaacacaggaggatcctacaacagctcagaccggggcagtagtacatctgggagtcaggggcacaagaaaggggcaagaacacccaaggtaccaaaacagggtggcatgaactgggcagacctgcttcctcctcccccagcacatcctcctccacacagcaatagcgaagagtacaacatttctgtagatgaaagctatgaccaagaaatgccatgtcccgtgccaccagcaaggatgtatttgcaacaagatgaattagaagaggaggaagatgaacgaggccccactccccctgttcggggagcagcttcttctccagctgccgtgtcctatagccatcagtccactgccactctgactccctccccacaggaagaactccagcccatgttacaggattgtccagaggagactggccacatgcagcaccagcccgacaggagacggcagcctgtgagtcctcctccaccaccacggccgatctcccctccacatacctatggctacatttcaggacccctggtctcagatatggatacggatgcgccagaagaggaagaagacgaagccgacatggaggtagccaagatgcaaaccagaaggcttttgttacgtgggcttgagcagacacctgcctccagtgttggggacctggagagctctgtcacggggtccatgatcaacggctggggctcagcctcagaggaggacaacatttccagcggacgctccagtgttagttcttcggacggctcctttttcactgatgctgactttgcccaggcagtcgcagcagcggcagagtatgctggtctgaaagtagcacgacggcaaatgcaggatgctgctggtcgtcgacattttcatgcgtctcagtgccctaggcccacaagtcccgtgtctacagacagcaacatgagtgccgccgtaatgcagaaaaccagaccagccaagaaactgaaacaccagccaggacatctgcgcagagaaacctacacagatgatcttccaccacctcctgtgccgccacctgctataaagtcacctactgcccaatccaagacacagctggaagtacgacctgtagtggtgccaaaactcccttctatggatgcaagaacagacagatcatcagacagaaaaggaagcagttacaaggggagagaagtgttggatggaagacaggttgttgacatgcgaacaaatccaggtgatcccagagaagcacaggaacagcaaaatgacgggaaaggacgtggaaacaaggcagcaaaacgagaccttccaccagcaaagactcatctcatccaagaggatattctaccttattgtagacctacttttccaacatcaaataatcccagagatcccagttcctcaagctcaatgtcatcaagaggatcaggaagcagacaaagagaacaagcaaatgtaggtcgaagaaatattgcagaaatgcaggtacttggaggatatgaaagaggagaagataataatgaagaattagaggaaactgaaagctga

SEQ ID NO: 94 - DNA, 4956 bp, Homo sapiens
  source 1..4956: mol_type = other DNA
atgaaatggaaacatgttccttttttggtcatgatatcactcctcagcttatccccaaatcacctgtttctggcccagcttattccagaccctgaagatgtagagagggggaacgaccacgggacgccaatccccacctctgataacgatgacaattcgctgggctatacaggctcccgtcttcgtcaggaagattttccacctcgcattgttgaacacccttcagacctgattgtctcaaaaggagaacctgcaactttgaactgcaaagctgaaggccgccccacacccactattgaatggtacaaagggggagagagagtggagacagacaaagatgaccctcgctcacaccgaatgttgctgccgagtggatctttatttttcttacgtatagtacatggacggaaaagtagacctgatgaaggagtctatgtctgtgtagcaaggaattaccttggagaggctgtgagccacaatgcatcgctggaagtagccatacttcgggatgacttcagacaaaacccttcggatgtcatggttgcagtaggagagcctgcagtaatggaatgccaacctccacgaggccatcctgagcccaccatttcatggaagaaagatggctctccactggatgataaagatgaaagaataactatacgaggaggaaagctcatgatcacttacacccgtaaaagtgacgctggcaaatatgtttgtgttggtaccaatatggttggggaacgtgagagtgaagtagccgagctgactgtcttagagagaccatcatttgtgaagagacccagtaacttggcagtaactgtggatgacagtgcagaatttaaatgtgaggcccgaggtgaccctgtacctacagtacgatggaggaaagatgatggagagctgcccaaatccagatatgaaatccgagatgatcataccttgaaaattaggaaggtgacagctggtgacatgggttcatacacttgtgttgcagaaaatatggtgggcaaagctgaagcatctgctactctgactgttcaagaacctccacattttgttgtgaaaccccgtgaccaggttgttgctttgggacggactgtaacttttcagtgtgaagcaaccggaaatcctcaaccagctattttctggaggagagaagggagtcagaatctacttttctcatatcaaccaccacagtcatccagccgattttcagtctcccagactggcgacctcacaattactaatgtccagcgatctgatgttggttattacatctgccagactttaaatgttgctggaagcatcatcacaaaggcatatttggaagttacagatgtgattgcagatcggcctcccccagttattcgacaaggtcctgtgaatcagactgtagccgtggatggcactttcgtcctcagctgtgtggccacaggcagtccagtgcccaccattctgtggagaaaggatggagtcctcgtttcaacccaagactctcgaatcaaacagttggagaatggagtactgcagatccgatatgctaagctgggtgatactggtcggtacacctgcattgcatcaacccccagtggtgaagcaacatggagtgcttacattgaagttcaagaatttggagttccagttcagcctccaagacctactgacccaaatttaatccctagtgccccatcaaaacctgaagtgacagatgtcagcagaaatacagtcacattatcgtggcaaccaaatttgaattcaggagcaactccaacatcttatattatagaagccttcagccatgcatctggtagcagctggcagaccgtagcagagaatgtgaaaacagaaacatctgccattaaaggactcaaacctaatgcaatttaccttttccttgtgagggcagctaatgcatatggaattagtgatccaagccaaatatcagatccagtgaaaacacaagatgtcctaccaacaagtcagggggtggaccacaagcaggtccagagagagctgggaaatgctgttctgcacctccacaaccccaccgtcctttcttcctcttccatcgaagtgcactggacagtagatcaacagtctcagtatatacaaggatataaaattctctatcggccatctggagccaaccacggagaatcagactggttagtttttgaagtgaggacgccagccaaaaacagtgtggtaatccctgatctcagaaagggagtcaactatgaaattaaggctcgccctttttttaatgaatttcaaggagcagatagtgaaatcaagtttgccaaaaccctggaagaagcacccagtgccccaccccaaggtgtaactgtatccaagaatgatggaaacggaactgcaattctagttagttggcagccacctccagaagacactcaaaatggaatggtccaagagtataaggtttggtgtctgggcaatgaaactcgataccacatcaacaaaacagtggatggttccaccttttccgtggtcattccctttcttgttcctggaatccgatacagtgtggaagtggcagccagcactggggctgggtctggggtaaagagtgagcctcagttcatccagctggatgcccatggaaaccctgtgtcacctgaggaccaagtcagcctcgctcagcagatttcagatgtggtgaagcagccggccttcatagcaggtattggagcagcctgttggatcatcctcatggtcttcagcatctggctttatcgacaccgcaagaagagaaacggacttactagtacctacgcgggtatcagaaaagtcccgtcttttaccttcacaccaacagtaacttaccagagaggaggcgaagctgtcagcagtggagggaggcctggacttctcaacatcagtgaacctgccgcgcagccatggctggcagacacgtggcctaatactggcaacaaccacaatgactgctccatcagctgctgcacggcaggcaatggaaacagcgacagcaacctcactacctacagtcgcccagctgattgtatagcaaattataacaaccaactggataacaaacaaacaaatctgatgctccctgagtcaactgtttatggtgatgtggaccttagtaacaaaatcaatgagatgaaaaccttcaatagcccaaatctgaaggatgggcgttttgtcaatccatcagggcagcctactccttacgccaccactcagctcatccagtcaaacctcagcaacaacatgaacaatggcagcggggactctggcgagaagcactggaaaccactgggacagcagaaacaagaagtggcaccagttcagtacaacatcgtggagcaaaacaagctgaacaaagattatcgagcaaatgacacagttcctccaactatcccatacaaccaatcatacgaccagaacacaggaggatcctacaacagctcagaccggggcagtagtacatctgggagtcaggggcacaagaaaggggcaagaacacccaaggtaccaaaacagggtggcatgaactgggcagacctgcttcctcctcccccagcacatcctcctccacacagcaatagcgaagagtacaacatttctgtagatgaaagctatgaccaagaaatgccatgtcccgtgccaccagcaaggatgtatttgcaacaagatgaattagaagaggaggaagatgaacgaggccccactccccctgttcggggagcagcttcttctccagctgccgtgtcctatagccatcagtccactgccactctgactccctccccacaggaagaactccagcccatgttacaggattgtccagaggagactggccacatgcagcaccagcccgacaggagacggcagcctgtgagtcctcctccaccaccacggccgatctcccctccacatacctatggctacatttcaggacccctggtctcagatatggatacggatgcgccagaagaggaagaagacgaagccgacatggaggtagccaagatgcaaaccagaaggcttttgttacgtgggcttgagcagacacctgcctccagtgttggggacctggagagctctgtcacggggtccatgatcaacggctggggctcagcctcagaggaggacaacatttccagcggacgctccagtgttagttcttcggacggctcctttttcactgatgctgactttgcccaggcagtcgcagcagcggcagagtatgctggtctgaaagtagcacgacggcaaatgcaggatgctgctggccgtcgacattttcatgcgtctcagtgccctaggcccacaagtcccgtgtctacagacagcaacatgagtgccgccgtaatgcagaaaaccagaccagccaagaaactgaaacaccagccaggacatctgcgcagagaaacctacacagatgatcttccaccacctcctgtgccgccacctgctataaagtcacctactgcccaatccaagacacagctggaagtacgacctgtagtggtgccaaaactcccttctatggatgcaagaacagacagatcatcagacagaaaaggaagcagttacaaggggagagaagtgttggatggaagacaggttgttgacatgcgaacaaatccaggtgatcccagagaagcacaggaacagcaaaatgacgggaaaggacgtggaaacaaggcagcaaaacgagaccttccaccagcaaagactcatctcatccaagaggatattctaccttattgtagacctacttttccaacatcaaataatcccagagatcccagttcctcaagctcaatgtcatcaagaggatcaggaagcagacaaagagaacaagcaaatgtaggtcgaagaaatattgcagaaatgcaggtacttggaggatatgaaagaggagaagataataatgaagaattagaggaaactgaaagctga

SEQ ID NO: 95 - DNA, 2964 bp, Homo sapiens
  source 1..2964: mol_type = other DNA
atggagctccgggtgctgctctgctgggcttcgttggccgcagctttggaagagaccctgctgaacacaaaattggaaactgctgatctgaagtgggtgacattccctcaggtggacgggcagtgggaggaactgagcggcctggatgaggaacagcacagcgtgcgcacctacgaagtgtgtgacgtgcagcgtgccccgggccaggcccactggcttcgcacaggttgggtcccacggcggggcgccgtccacgtgtacgccacgctgcgcttcaccatgctcgagtgcctgtccctgcctcgggctgggcgctcctgcaaggagaccttcaccgtcttctactatgagagcgatgcggacacggccacggccctcacgccagcctggatggagaacccctacatcaaggtggacacggtggccgcggagcatctcacccggaagcgccctggggccgaggccaccgggaaggtgaatgtcaagacgctgcgtctgggaccgctcagcaaggctggcttctacctggccttccaggaccagggtgcctgcatggccctgctatccctgcacctcttctacaaaaagtgcgcccagctgactgtgaacctgactcgattcccggagactgtgcctcgggagctggttgtgcccgtggccggtagctgcgtggtggatgccgtccccgcccctggccccagccccagcctctactgccgtgaggatggccagtgggccgaacagccggtcacgggctgcagctgtgctccggggttcgaggcagctgaggggaacaccaagtgccgagcctgtgcccagggcaccttcaagcccctgtcaggagaagggtcctgccagccatgcccagccaatagccactctaacaccattggatcagccgtctgccagtgccgcgtcgggtacttccgggcacgcacagacccccggggtgcaccctgcaccacccctccttcggctccgcggagcgtggtttcccgcctgaacggctcctccctgcacctggaatggagtgcccccctggagtctggtggccgagaggacctcacctacgccctccgctgccgggagtgccgacccggaggctcctgtgcgccctgcgggggagacctgacttttgaccccggcccccgggacctggtggagccctgggtggtggttcgagggctacgtcctgacttcacctatacctttgaggtcactgcattgaacggggtatcctccttagccacggggcccgtcccatttgagcctgtcaatgtcaccactgaccgagaggtacctcctgcagtgtccgacatccgggtgacgcggtcctcacccagcagcttgagcctggcctgggctgttccccgggcacccagtggggctgtgctggactacgaggtcaaataccatgagaagggcgccgagggtcccagcagcgtgcggttcctgaagacgtcagaaaaccgggcagagctgcgggggctgaagcggggagccagctacctggtgcaggtacgggcgcgctctgaggccggctacgggcccttcggccaggaacatcacagccagacccaactggatgagagcgagggctggcgggagcagctggccctgattgcgggcacggcagtcgtgggtgtggtcctggtcctggtggtcattgtggtcgcagttctctgcctcaggaagcagagcaatgggagagaagcagaatattcggacaaacacggacagtatctcatcgggcatggtactaaggtctacatcgaccccttcacttatgaagaccctaatgaggctgtgagggaatttgcaaaagagatcgatgtctcctacgtcaagattgaagaggtgattggtgcaggtgagtttggcgaggtgtgccgggggcggctcaaggccccagggaagaaggagagctgtgtggcaatcaagaccctgaagggtggctacacggagcggcagcggcgtgagtttctgagcgaggcctccatcatgggccagttcgagcaccccaatatcatccgcctggagggcgtggtcaccaacagcatgcccgtcatgattctcacagagttcatggagaacggcgccctggactccttcctgcggctaaacgacggacagttcacagtcatccagctcgtgggcatgctgcggggcatcgcctcgggcatgcggtaccttgccgagatgagctacgtccaccgagacctggctgctcgcaacatcctagtcaacagcaacctcgtctgcaaagtgtctgactttggcctttcccgattcctggaggagaactcttccgatcccacctacacgagctccctgggaggaaagattcccatccgatggactgccccggaggccattgccttccggaagttcacttccgccagtgatgcctggagttacgggattgtgatgtgggaggtgatgtcatttggggagaggccgtactgggacatgagcaatcaggacgtgatcaatgccattgaacaggactaccggctgcccccgcccccagactgtcccacctccctccaccagctcatgctggactgttggcagaaagaccggaatgcccggccccgcttcccccaggtggtcagcgccctggacaagatgatccggaaccccgccagcctcaaaatcgtggcccgggagaatggcggggcctcacaccctctcctggaccagcggcagcctcactactcagcttttggctctgtgggcgagtggcttcgggccatcaaaatgggaagatacgaagaaagtttcgcagccgctggctttggctccttcgagctggtcagccagatctctgctgaggacctgctccgaatcggagtcactctggcgggacaccagaagaaaatcttggccagtgtccagcacatgaagtcccaggccaagccgggaaccccgggtgggacaggaggaccggccccgcagtactga

SEQ ID NO: 96 - DNA, 636 bp, Homo sapiens
  source 1..636: mol_type = other DNA
atggccaacgcggggctgcagctgttgggcttcattctcgccttcctgggatggatcggcgccatcgtcagcactgccctgccccagtggaggatttactcctatgccggcgacaacatcgtgaccgcccaggccatgtacgaggggctgtggatgtcctgcgtgtcgcagagcaccgggcagatccagtgcaaagtctttgactccttgctgaatctgagcagcacattgcaagcaacccgtgccttgatggtggttggcatcctcctgggagtgatagcaatctttgtggccaccgttggcatgaagtgtatgaagtgcttggaagacgatgaggtgcagaagatgaggatggctgtcattgggggtgcgatatttcttcttgcaggtctggctattttagttgccacagcatggtatggcaatagaatcgttcaagaattctatgaccctatgaccccagtcaatgccaggtacgaatttggtcaggctctcttcactggctgggctgctgcttctctctgccttctgggaggtgccctactttgctgttcctgtccccgaaaaacaacctcttacccaacaccaaggccctatccaaaacctgcaccttccagcgggaaagactacgtgtga

SEQ ID NO: 97 - DNA, 1524 bp, Homo sapiens
  source 1..1524: mol_type = other DNA
atggcgggtgcgggcccgaagcggcgcgcgctagcggcgccggcggccgaggagaaggaagaggcgcgggagaagatgctggccgccaagagcgcggacggctcggcgccggcaggcgagggcgagggcgtgaccctgcagcggaacatcacgctgctcaacggcgtggccatcatcgtggggaccattatcggctcgggcatcttcgtgacgcccacgggcgtgctcaaggaggcaggctcgccggggctggcgctggtggtgtgggccgcgtgcggcgtcttctccatcgtgggcgcgctctgctacgcggagctcggcaccaccatctccaaatcgggcggcgactacgcctacatgctggaggtctacggctcgctgcccgccttcctcaagctctggatcgagctgctcatcatccggccttcatcgcagtacatcgtggccctggtcttcgccacctacctgctcaagccgctcttccccacctgcccggtgcccgaggaggcagccaagctcgtggcctgcctctgcgtgctgctgctcacggccgtgaactgctacagcgtgaaggccgccacccgggtccaggatgcctttgccgccgccaagctcctggccctggccctgatcatcctgctgggcttcgtccagatcgggaagggtgatgtgtccaatctagatcccaacttctcatttgaaggcaccaaactggatgtggggaacattgtgctggcattatacagcggcctctttgcctatggaggatggaattacttgaatttcgtcacagaggaaatgatcaacccctacagaaacctgcccctggccatcatcatctccctgcccatcgtgacgctggtgtacgtgctgaccaacctggcctacttcaccaccctgtccaccgagcagatgctgtcgtccgaggccgtggccgtggacttcgggaactatcacctgggcgtcatgtcctggatcatccccgtcttcgtgggcctgtcctgcttcggctccgtcaatgggtccctgttcacatcctccaggctcttcttcgtggggtcccgggaaggccacctgccctccatcctctccatgatccacccacagctcctcacccccgtgccgtccctcgtgttcacgtgtgtgatgacgctgctctacgccttctccaaggacatcttctccgtcatcaacttcttcagcttcttcaactggctctgcgtggccctggccatcatcggcatgatctggctgcgccacagaaagcctgagcttgagcggcccatcaaggtgaacctggccctgcctgtgttcttcatcctggcctgcctcttcctgatcgccgtctccttctggaagacacccgtggagtgtggcatcggcttcaccatcatcctcagcgggctgcccgtctacttcttcggggtctggtggaaaaacaagcccaagtggctcctccagggcatcttctccacgaccgtcctgtgtcagaagctcatgcaggtggtcccccaggagacatag

SEQ ID NO: 98 - DNA, 1830 bp, Homo sapiens
  source 1..1830: mol_type = other DNA
atgaagtgggtggaatcaatttttttaattttcctactaaattttactgaatccagaacactgcatagaaatgaatatggaatagcttccatattggattcttaccaatgtactgcagagataagtttagctgacctggctaccatattttttgcccagtttgttcaagaagccacttacaaggaagtaagcaaaatggtgaaagatgcattgactgcaattgagaaacccactggagatgaacagtcttcagggtgtttagaaaaccagctacctgcctttctggaagaactttgccatgagaaagaaattttggagaagtacggacattcagactgctgcagccaaagtgaagagggaagacataactgttttcttgcacacaaaaagcccactccagcatcgatcccacttttccaagttccagaacctgtcacaagctgtgaagcatatgaagaagacagggagacattcatgaacaaattcatttatgagatagcaagaaggcatcccttcctgtatgcacctacaattcttctttgggctgctcgctatgacaaaataattccatcttgctgcaaagctgaaaatgcagttgaatgcttccaaacaaaggcagcaacagttacaaaagaattaagagaaagcagcttgttaaatcaacatgcatgtgcagtaatgaaaaattttgggacccgaactttccaagccataactgttactaaactgagtcagaagtttaccaaagttaattttactgaaatccagaaactagtcctggatgtggcccatgtacatgagcactgttgcagaggagatgtgctggattgtctgcaggatggggaaaaaatcatgtcctacatatgttctcaacaagacactctgtcaaacaaaataacagaatgctgcaaactgaccacgctggaacgtggtcaatgtataattcatgcagaaaatgatgaaaaacctgaaggtctatctccaaatctaaacaggtttttaggagatagagattttaaccaattttcttcaggggaaaaaaatatcttcttggcaagttttgttcatgaatattcaagaagacatcctcagcttgctgtctcagtaattctaagagttgctaaaggataccaggagttattggagaagtgtttccagactgaaaaccctcttgaatgccaagataaaggagaagaagaattacagaaatacatccaggagagccaagcattggcaaagcgaagctgcggcctcttccagaaactaggagaatattacttacaaaatgcgtttctcgttgcttacacaaagaaagccccccagctgacctcgtcggagctgatggccatcaccagaaaaatggcagccacagcagccacttgttgccaactcagtgaggacaaactattggcctgtggcgagggagcggctgacattattatcggacacttatgtatcagacatgaaatgactccagtaaaccctggtgttggccagtgctgcacttcttcatatgccaacaggaggccatgcttcagcagcttggtggtggatgaaacatatgtccctcctgcattctctgatgacaagttcattttccataaggatctgtgccaagctcagggtgtagcgctgcaaacgatgaagcaagagtttctcattaaccttgtgaagcaaaagccacaaataacagaggaacaacttgaggctgtcattgcagatttctcaggcctgttggagaaatgctgccaaggccaggaacaggaagtctgctttgctgaagagggacaaaaactgatttcaaaaactcgtgctgctttgggagtttaa

SEQ ID NO: 99 - DNA, 2052 bp, Homo sapiens
  source 1..2052: mol_type = other DNA
atggcgctcttcgtgcggctgctggctctcgccctggctctggccctgggccccgccgcgaccctggcgggtcccgccaagtcgccctaccagctggtgctgcagcacagcaggctccggggccgccagcacggccccaacgtgtgtgctgtgcagaaggttattggcactaataggaagtacttcaccaactgcaagcagtggtaccaaaggaaaatctgtggcaaatcaacagtcatcagctacgagtgctgtcctggatatgaaaaggtccctggggagaagggctgtccagcagccctaccactctcaaacctttacgagaccctgggagtcgttggatccaccaccactcagctgtacacggaccgcacggagaagctgaggcctgagatggaggggcccggcagcttcaccatcttcgcccctagcaacgaggcctgggcctccttgccagctgaagtgctggactccctggtcagcaatgtcaacattgagctgctcaatgccctccgctaccatatggtgggcaggcgagtcctgactgatgagctgaaacacggcatgaccctcacctctatgtaccagaattccaacatccagatccaccactatcctaatgggattgtaactgtgaactgtgcccggctcctgaaagccgaccaccatgcaaccaacggggtggtgcacctcatcgataaggtcatctccaccatcaccaacaacatccagcagatcattgagatcgaggacacctttgagacccttcgggctgctgtggctgcatcagggctcaacacgatgcttgaaggtaacggccagtacacgcttttggccccgaccaatgaggccttcgagaagatccctagtgagactttgaaccgtatcctgggcgacccagaagccctgagagacctgctgaacaaccacatcttgaagtcagctatgtgtgctgaagccatcgttgcggggctgtctgtagagaccctggagggcacgacactggaggtgggctgcagcggggacatgctcactatcaacgggaaggcgatcatctccaataaagacatcctagccaccaacggggtgatccactacattgatgagctactcatcccagactcagccaagacactatttgaattggctgcagagtctgatgtgtccacagccattgaccttttcagacaagccggcctcggcaatcatctctctggaagtgagcggttgaccctcctggctcccctgaattctgtattcaaagatggaacccctccaattgatgcccatacaaggaatttgcttcggaaccacataattaaagaccagctggcctctaagtatctgtaccatggacagaccctggaaactctgggcggcaaaaaactgagagtttttgtttatcgtaatagcctctgcattgagaacagctgcatcgcggcccacgacaagagggggaggtacgggaccctgttcacgatggaccgggtgctgacccccccaatggggactgtcatggatgtcctgaagggagacaatcgctttagcatgctggtagctgccatccagtctgcaggactgacggagaccctcaaccgggaaggagtctacacagtctttgctcccacaaatgaagccttccgagccctgccaccaagagaacggagcagactcttgggagatgccaaggaacttgccaacatcctgaaataccacattggtgatgaaatcctggttagcggaggcatcggggccctggtgcggctaaagtctctccaaggtgacaagctggaagtcagcttgaaaaacaatgtggtgagtgtcaacaaggagcctgttgccgagcctgacatcatggccacaaatggcgtggtccatgtcatcaccaatgttctgcagcctccagccaacagacctcaggaaagaggggatgaacttgcagactctgcgcttgagatcttcaaacaagcatcagcgttttccagggcttcccagaggtctgtgcgactagcccctgtctatcaaaagttattagagaggatgaagcattag

SEQ ID NO: 100 - DNA, 912 bp, Homo sapiens
  source 1..912: mol_type = other DNA
atgagggcctggatcttctttctcctttgcctggccgggagggccttggcagcccctcagcaagaagccctgcctgatgagacagaggtggtggaagaaactgtggcagaggtgactgaggtatctgtgggagctaatcctgtccaggtggaagtaggagaatttgatgatggtgcagaggaaaccgaagaggaggtggtggcggaaaatccctgccagaaccaccactgcaaacacggcaaggtgtgcgagctggatgagaacaacacccccatgtgcgtgtgccaggaccccaccagctgcccagcccccattggcgagtttgagaaggtgtgcagcaatgacaacaagaccttcgactcttcctgccacttctttgccacaaagtgcaccctggagggcaccaagaagggccacaagctccacctggactacatcgggccttgcaaatacatccccccttgcctggactctgagctgaccgaattccccctgcgcatgcgggactggctcaagaacgtcctggtcaccctgtatgagagggatgaggacaacaaccttctgactgagaagcagaagctgcgggtgaagaagatccatgagaatgagaagcgcctggaggcaggagaccaccccgtggagctgctggcccgggacttcgagaagaactataacatgtacatcttccctgtacactggcagttcggccagctggaccagcaccccattgacgggtacctctcccacaccgagctggctccactgcgtgctcccctcatccccatggagcattgcaccacccgctttttcgagacctgtgacctggacaatgacaagtacatcgccctggatgagtgggccggctgcttcggcatcaagcagaaggatatcgacaaggatcttgtgatctaa

SEQ ID NO: 101 - DNA, 2292 bp, Homo sapiens
  source 1..2292: mol_type = other DNA
atgaaaactagcccccgtcggccactgattctcaaaagacggaggctgccccttcctgttcaaaatgccccaagtgaaacatcagaggaggaacctaagagatcccctgcccaacaggagtctaatcaagcagaggcctccaaggaagtggcagagtccaactcttgcaagtttccagctgggatcaagattattaaccaccccaccatgcccaacacgcaagtagtggccatccccaacaatgctaatattcacagcatcatcacagcactgactgccaagggaaaagagagtggcagtagtgggcccaacaaattcatcctcatcagctgtgggggagccccaactcagcctccaggactccggcctcaaacccaaaccagctatgatgccaaaaggacagaagtgaccctggagaccttgggaccaaaacctgcagctagggatgtgaatcttcctagaccacctggagccctttgcgagcagaaacgggagacctgtgcagatggtgaggcagcaggctgcactatcaacaatagcctatccaacatccagtggcttcgaaagatgagttctgatggactgggctcccgcagcatcaagcaagagatggaggaaaaggagaattgtcacctggagcagcgacaggttaaggttgaggagccttcgagaccatcagcgtcctggcagaactctgtgtctgagcggccaccctactcttacatggccatgatacaattcgccatcaacagcactgagaggaagcgcatgactttgaaagacatctatacgtggattgaggaccactttccctactttaagcacattgccaagccaggctggaagaactccatccgccacaacctttccctgcacgacatgtttgtccgggagacgtctgccaatggcaaggtctccttctggaccattcaccccagtgccaaccgctacttgacattggaccaggtgtttaagccactggacccagggtctccacaattgcccgagcacttggaatcacagcagaaacgaccgaatccagagctccgccggaacatgaccatcaaaaccgaactccccctgggcgcacggcggaagatgaagccactgctaccacgggtcagctcatacctggtacctatccagttcccggtgaaccagtcactggtgttgcagccctcggtgaaggtgccattgcccctggcggcttccctcatgagctcagagcttgcccgccatagcaagcgagtccgcattgcccccaaggtgctgctagctgaggaggggatagctcctctttcttctgcaggaccagggaaagaggagaaactcctgtttggagaagggttttctcctttgcttccagttcagactatcaaggaggaagaaatccagcctggggaggaaatgccacacttagcgagacccatcaaagtggagagccctcccttggaagagtggccctccccggccccatctttcaaagaggaatcatctcactcctgggaggattcgtcccaatctcccaccccaagacccaagaagtcctacagtgggcttaggtccccaacccggtgtgtctcggaaatgcttgtgattcaacacagggagaggagggagaggagccggtctcggaggaaacagcatctactgcctccctgtgtggatgagccggagctgctcttctcagaggggcccagtacttcccgctgggccgcagagctcccgttcccagcagactcctctgaccctgcctcccagctcagctactcccaggaagtgggaggaccttttaagacacccattaaggaaacgctgcccatctcctccaccccgagcaaatctgtcctccccagaacccctgaatcctggaggctcacgcccccagccaaagtagggggactggatttcagcccagtacaaaccccccagggtgcctctgaccccttgcctgaccccctggggctgatggatctcagcaccactcccttgcaaagtgctcccccccttgaatcaccgcaaaggctcctcagttcagaacccttagacctcatctccgtcccctttggcaactcttctccctcagatatagacgtccccaagccaggctccccggagccacaggtttctggccttgcagccaatcgttctctgacagaaggcctggtcctggacacaatgaatgacagcctcagcaagatcctgctggacatcagctttcctggcctggacgaggacccactgggccctgacaacatcaactggtcccagtttattcctgagctacagtag

SEQ ID NO: 102 - DNA, 2577 bp, Homo sapiens
  source 1..2577: mol_type = other DNA
atgtcggtggtggggttggacgtgggctcgcagagctgctacatcgcggtagcccgggccgggggcatcgagaccatcgccaatgagttcagcgaccggtgcaccccgtcagtcatatcatttggatcaaaaaatagaacaatcggagttgcagccaaaaatcagcaaatcactcatgcaaacaatacggtgtctaacttcaaaagatttcatggccgagcattcaatgaccccttcattcaaaaggagaaggaaaacttgagttacgatttggttccattgaaaaatggtggagttggaataaaggtaatgtacatgggtgaagaacatctatttagtgtggagcagataacagccatgttgttgactaagctgaaggaaactgctgaaaacagcctcaagaaaccagtaacagattgtgttatttcagtcccctccttctttacagatgctgagaggcgatctgtgttagatgctgcacagattgttggcctaaactgtttaagacttatgaatgacatgacagctgttgctttgaattacggaatttataagcaggatctcccaagcctggatgagaaacctcggatagtggtttttgttgatatgggacattcagcttttcaagtgtctgcttgtgcttttaacaagggaaaattgaaggtactgggaacagcttttgatcctttcttaggaggaaaaaacttcgatgaaaagttagtggaacatttttgtgcagaatttaaaactaagtacaagttggatgcaaaatccaaaatacgagcactcctacgtctgtatcaggaatgtgaaaaactgaaaaagctaatgagctctaacagcacagaccttccactgaatatcgaatgctttatgaatgataaagatgtttccggaaagatgaacaggtcacaatttgaagaactctgtgctgaacttctgcaaaagatagaagtacccctttattcactgttggaacaaactcatctcaaagtagaagatgtgagtgcagttgagattgttggaggcgctacacgaattccagctgtgaaggaaagaattgccaaattctttggaaaagatattagcacaacactcaatgcagatgaagcagtagccagaggatgtgcattacagtgtgcaatactttccccggcatttaaagttagagaattttccgtcacagatgcagttccttttccaatatctctgatctggaaccatgattcagaagatactgaaggtgttcatgaagtctttagtcgaaaccatgctgctcctttctccaaagttctcacctttctgagaagggggccttttgagctagaagctttctattctgatccccaaggagttccatatccagaagcaaaaataggccgctttgtagttcagaatgtttctgcacagaaagatggagaaaaatctagagtaaaagtcaaagtgcgagtcaacacccatggcattttcaccatctctacggcatctatggtggagaaagtcccaactgaggagaatgaaatgtcttctgaagctgacatggagtgtctgaatcagagaccaccagaaaacccagacactgataaaaatgtccagcaagacaacagtgaagctggaacacagccccaggtacaaactgatgctcaacaaacctcacagtctcccccttcacctgaacttacctcagaagaaaacaaaatcccagatgctgacaaagcaaatgaaaaaaaagttgaccagcctccagaagctaaaaagcccaaaataaaggtggtgaatgttgagctgcctattgaagccaacttggtctggcagttagggaaagaccttcttaacatgtatattgagacagagggtaagatgataatgcaagataaattggaaaaagaaaggaatgatgctaaaaatgcagttgaggaatatgtgtatgagttcagagacaagctgtgtggaccatatgaaaaatttatatgtgagcaggatcatcaaaattttttgagactcctcacagaaactgaagactggctgtatgaagaaggagaggaccaagctaaacaagcatatgttgacaagttggaagaattaatgaaaattggcactccagttaaagttcggtttcaggaagctgaagaacggccaaaaatgtttgaagaactaggacagaggctgcagcattatgccaagatagcagctgacttcagaaataaggatgagaaatacaaccatattgatgagtctgaaatgaaaaaagtggagaagtctgttaatgaagtgatggaatggatgaataatgtcatgaatgctcaggctaaaaagagtcttgatcaggatccagttgtacgtgctcaggaaattaaaacaaaaatcaaggaattgaacaacacatgtgaacccgttgtaacacaaccgaaaccaaaaattgaatcacccaaactggaaagaactccaaatggcccaaatattgataaaaaggaagaagatttagaagacaaaaacaattttggtgctgaacctccacatcagaatggtgaatgttaccctaatgagaaaaattctgttaatatggacttggactag

SEQ ID NO: 103 - protein, 135 aa, Homo sapiens
MMKSLRVLLVILWLQLSWVWSQQKEVEQDPGPLSVPEGAIVSLNCTYSNSAFQYFMWYRQYSRKGPELLMYTYSSGNKEDGRFTAQVDKSSKYISLFIRDSQPSDSATYLCAQRIVMEYGNKLVFGAGTILRVKS

SEQ ID NO: 104 - protein, 130 aa, Homo sapiens
MDTWLVCWAIFSLLKAGLTEPEVTQTPSHQVTQMGQEVILRCVPISNHLYFYWYRQILGQKVEFLVSFYNNEISEKSEIFDDQFSVERPDGSNFTLKIRSTKLEDSAMYFCASSEGAEAFFGQGTRLTVV

SEQ ID NO: 105 - protein, 132 aa, Homo sapiens
MKSLRVLLVILWLQLSWVWSQQKEVEQNSGPLSVPEGAIASLNCTYSDRGSQSFFWYRQYSGKSPELIMFIYSNGDKEDGRFTAQLNKASQYVSLLIRDSQPSDSATYLCAVNMDGNNRLAFGKGNQVVVIP

SEQ ID NO: 106 - protein, 137 aa, Homo sapiens
MRSWPGPEMGTRLFFYVALCLLWTGHMDAGITQSPRHKVTETGTPVTLRCHQTENHRYMYWYRQDPGHGLRLIHYSYGVKDTDKGEVSDGYSVSRSKTEDFLLTLESATSSQTSVYFCASVYGSEAFFGQGTRLTVV

SEQ ID NO: 107 - protein, 133 aa, Homo sapiens
MASAPISMLAMLFTLSGLRAQSVAQPEDQVNVAEGNPLTVKCTYSVSGNPYLFWYVQYPNRGLQFLLKYITGDNLVKGSYGFEAEFNKSQTSFHLKKPSALVSDSALYFCAVNPTGGGNKLTFGTGTQLKVEL

SEQ ID NO: 108 - protein, 132 aa, Homo sapiens
MATRLLCCVVLCLLGEELIDARVTQTPRDKVTEMGQEVTMRCQPILGHNTVFWYRQTMMQGLELLAYFRNRAPLDDSGMPKDRFSAEMPDATLATLKIQPSEPRDSAVYFCASGLGGNQPQHFGDGTRLSIL

SEQ ID NO: 109 - protein, 132 aa, Homo sapiens
MKSLRVLLVILWLQLSWVWSQQKEVEQNSGPLSVPEGAIASLNCTYSDRGSQSFFWYRQYSGKSPELIMFIYSNGDKEDGRFTAQLNKASQYVSLLIRDSQPSDSATYLCAVKGTGRRALTFGSGTRLQVQP

SEQ ID NO: 110 - protein, 133 aa, Homo sapiens
MGCRLLCCAVLCLLGAVPIDTEVTQTPKHLVMGMTNKKSLKCEQHMGHRAMYWYKQKAKKPPELMFVYSYEKLSINESVPSRFSPECPNSSLLNLHLHALQPEDSALYLCASSQSGVGNTEAFFGQGTRLTVV

SEQ ID NO: 111 - protein, 133 aa, Homo sapiens
MLLELIPLLGIHFVLRTARAQSVTQPDIHITVSEGASLELRCNYSYGATPYLFWYVQSPGQGLQLLLKYFSGDTLVQGIKGFEAEFKRSQSSFNLRKPSVHWSDAAEYFCAVGSPSGYSTLTFGKGTMLLVSP

SEQ ID NO: 112 - protein, 131 aa, Homo sapiens
MGPQLLGYVVLCLLGAGPLEAQVTQNPRYLITVTGKKLTVTCSQNMNHEYMSWYRQDPGLGLRQIYYSMNVEVTDKGDVPEGYKVSRKEKRNFPLILESPSPNQTSLYFCASSPTRFYEQYFGPGTRLTVT

SEQ ID NO: 113 - DNA, 405 bp, Homo sapiens
  source 1..405: mol_type = other DNA
atgatgaaatccttgagagttttactggtgatcctgtggcttcagttaagctgggtttggagccaacagaaggaggtggagcaggatcctggaccactcagtgttccagagggagccattgtttctctcaactgcacttacagcaacagtgcttttcaatacttcatgtggtacagacagtattccagaaaaggccctgagttgctgatgtacacatactccagtggtaacaaagaagatggaaggtttacagcacaggtcgataaatccagcaagtatatctccttgttcatcagagactcacagcccagtgattcagccacctacctctgtgcccaaagaattgtcatggaatatggaaacaagctggtctttggcgcaggaaccattctgagagtcaagtcc

SEQ ID NO: 114 - DNA, 390 bp, Homo sapiens
  source 1..390: mol_type = other DNA
atggatacctggctcgtatgctgggcaatttttagtctcttgaaagcaggactcacagaacctgaagtcacccagactcccagccatcaggtcacacagatgggacaggaagtgatcttgcgctgtgtccccatctctaatcacttatacttctattggtacagacaaatcttggggcagaaagtcgagtttctggtttccttttataataatgaaatctcagagaagtctgaaatattcgatgatcaattctcagttgaaaggcctgatggatcaaatttcactctgaagatccggtccacaaagctggaggactcagccatgtacttctgtgccagcagtgagggggctgaagctttctttggacaaggcaccagactcacagttgta

SEQ ID NO: 115 - DNA, 396 bp, Homo sapiens
  source 1..396: mol_type = other DNA
atgaaatccttgagagttttactagtgatcctgtggcttcagttgagctgggtttggagccaacagaaggaggtggagcagaattctggacccctcagtgttccagagggagccattgcctctctcaactgcacttacagtgaccgaggttcccagtccttcttctggtacagacaatattctgggaaaagccctgagttgataatgttcatatactccaatggtgacaaagaagatggaaggtttacagcacagctcaataaagccagccagtatgtttctctgctcatcagagactcccagcccagtgattcagccacctacctctgtgccgtgaacatggacgggaacaacagactcgcttttgggaaggggaaccaagtggtggtcatacca

SEQ ID NO: 116 - DNA, 411 bp, Homo sapiens
  source 1..411: mol_type = other DNA
atgagatcctggcctggacctgaaatgggcacaaggttgttcttctatgtggccctttgtctcctgtggacaggacacatggatgctggaatcacccagagcccaagacacaaggtcacagagacaggaacaccagtgactctgagatgtcatcagactgagaaccaccgctatatgtactggtatcgacaagacccggggcatgggctgaggctgatccattactcatatggtgttaaagatactgacaaaggagaagtctcagatggctatagtgtctctagatcaaagacagaggatttcctcctcactctggagtccgctaccagctcccagacatctgtgtacttctgtgccagcgtttacgggtctgaagctttctttggacaaggcaccagactcacagttgta

SEQ ID NO: 117 - DNA, 399 bp, Homo sapiens
  source 1..399: mol_type = other DNA
atggcctctgcacccatctcgatgcttgcgatgctcttcacattgagtgggctgagagctcagtcagtggctcagccggaagatcaggtcaacgttgctgaagggaatcctctgactgtgaaatgcacctattcagtctctggaaacccttatcttttttggtatgttcaataccccaaccgaggcctccagttccttctgaaatacatcacaggggataacctggttaaaggcagctatggctttgaagctgaatttaacaagagccaaacctccttccacctgaagaaaccatctgcccttgtgagcgactccgctttgtacttctgtgctgtgaaccccacgggaggaggaaacaaactcacctttgggacaggcactcagctaaaagtggaactc

SEQ ID NO: 118 - DNA, 396 bp, Homo sapiens
  source 1..396: mol_type = other DNA
atggccaccaggctcctctgctgtgtggttctttgtctcctgggagaagagcttatagatgctagagtcacccagacaccaagggacaaggtgacagagatgggacaagaagtaacaatgagatgtcagccaattttaggccacaatactgttttctggtacagacagaccatgatgcaaggactggagttgctggcttacttccgcaaccgggctcctctagatgattcggggatgccgaaggatcgattctcagcagagatgcctgatgcaactttagccactctgaagatccagccctcagaacccagggactcagctgtgtatttttgtgctagtggtttggggggaaatcagccccagcattttggtgatgggactcgactctccatccta

SEQ ID NO: 119 - DNA, 396 bp, Homo sapiens
  source 1..396: mol_type = other DNA
atgaaatccttgagagttttactagtgatcctgtggcttcagttgagctgggtttggagccaacagaaggaggtggagcagaattctggacccctcagtgttccagagggagccattgcctctctcaactgcacttacagtgaccgaggttcccagtccttcttctggtacagacaatattctgggaaaagccctgagttgataatgttcatatactccaatggtgacaaagaagatggaaggtttacagcacagctcaataaagccagccagtatgtttctctgctcatcagagactcccagcccagtgattcagccacctacctctgtgccgtgaaggggacgggcaggagagcacttacttttgggagtggaacaagactccaagtgcaacca

SEQ ID NO: 120 - DNA, 399 bp, Homo sapiens
  source 1..399: mol_type = other DNA
atgggctgcaggctgctctgctgtgcggttctctgtctcctgggagcagttcccatagacactgaagttacccagacaccaaaacacctggtcatgggaatgacaaataagaagtctttgaaatgtgaacaacatatggggcacagggctatgtattggtacaagcagaaagctaagaagccaccggagctcatgtttgtctacagctatgagaaactctctataaatgaaagtgtgccaagtcgcttctcacctgaatgccccaacagctctctcttaaaccttcacctacacgccctgcagccagaagactcagccctgtatctctgcgccagcagccaaagtggggtcgggaacactgaagctttctttggacaaggcaccagactcacagttgta

SEQ ID NO: 121 - DNA, 399 bp, Homo sapiens
  source 1..399: mol_type = other DNA
atgctcctggagcttatcccactgctggggatacattttgtcctgagaactgccagagcccagtcagtgacccagcctgacatccacatcactgtctctgaaggagcctcactggagttgagatgtaactattcctatggggcaacaccttatctcttctggtatgtccagtcccccggccaaggcctccagctgctcctgaagtacttttcaggagacactctggttcaaggcattaaaggctttgaggctgaatttaagaggagtcaatcttccttcaatctgaggaaaccctctgtgcattggagtgatgctgctgagtacttctgtgctgtgggttcgccttcaggatacagcaccctcacctttgggaaggggactatgcttctagtctctcca

SEQ ID NO: 122 - DNA, 393 bp, Homo sapiens
  source 1..393: mol_type = other DNA
atgggcccccagctccttggctatgtggtcctttgccttctaggagcaggccccctggaagcccaagtgacccagaacccaagatacctcatcacagtgactggaaagaagttaacagtgacttgttctcagaatatgaaccatgagtatatgtcctggtatcgacaagacccagggctgggcttaaggcagatctactattcaatgaatgttgaggtgactgataagggagatgttcctgaagggtacaaagtctctcgaaaagagaagaggaatttccccctgatcctggagtcgcccagccccaaccagacctctctgtacttctgtgccagcagccccactaggttctacgagcagtacttcgggccgggcaccaggctcacggtcaca

SEQ ID NO: 123 - protein, 129 aa, Homo sapiens
MVLKFSVSILWIQLAWVSTQLLEQSPQFLSIQEGENLTVYCNSSSVFSSLQWYRQEPGEGPVLLVTVVTGGEVKKLKRLTFQFGDARKDSSLHITAAQPGDTGLYLCAGRYSSASKIIFGSGTRLSIRP

SEQ ID NO: 124 - protein, 133 aa, Homo sapiens
MGFRLLCCVAFCLLGAGPVDSGVTQTPKHLITATGQRVTLRCSPRSGDLSVYWYQQSLDQGLQFLIQYYNGEERAKGNILERFSAQQFPDLHSELNLSSLELGDSALYFCASSVGGGAPNEQFFGPGTRLTVL

SEQ ID NO: 125 - protein, 128 aa, Homo sapiens
METLLGLLILWLQLQWVSSKQEVTQIPAALSVPEGENLVLNCSFTDSAIYNLQWFRQDPGKGLTSLLLIQSSQREQTSGRLNASLDKSSGRSTLYIAASQPGDSATYLCAVTRRALTFGSGTRLQVQP

SEQ ID NO: 126 - protein, 135 aa, Homo sapiens
MGSRLLCWVLLCLLGAGPVKAGVTQTPRYLIKTRGQQVTLSCSPISGHRSVSWYQQTPGQGLQFLFEYFSETQRNKGNFPGRFSGRQFSNSRSEMNVSTLELGDSALYLCASSVTSGRTHTDTQYFGPGTRLTVL

SEQ ID NO: 127 - protein, 131 aa, Homo sapiens
MMISLRVLLVILWLQLSWVWSQRKEVEQDPGPFNVPEGATVAFNCTYSNSASQSFFWYRQDCRKEPKLLMSVYSSGNEDGRFTAQLNRASQYISLLIRDSKLSDSATYLCKISGGYNKLIFGAGTRLAVHP

SEQ ID NO: 128 - protein, 133 aa, Homo sapiens
MGFRLLCCVAFCLLGAGPVDSGVTQTPKHLITATGQRVTLRCSPRSGDLSVYWYQQSLDQGLQFLIQYYNGEERAKGNILERFSAQQFPDLHSELNLSSLELGDSALYFCASSVGGGLGTEAFFGQGTRLTVV

SEQ ID NO: 129 - protein, 127 aa, Homo sapiens
MRQVARVIVFLTLSTLSLAKTTQPISMDSYEGQEVNITCSHNNIATNDYITWYQQFPSQGPRFIIQGYKTKVTNEVASLFIPADRKSSTLSLPRVSLSDTAVYYCLVGHSGNTPLVFGKGTRLSVIA

SEQ ID NO: 130 - protein, 130 aa, Homo sapiens
MISLRVLLVILWLQLSWVWSQRKEVEQDPGPFNVPEGATVAFNCTYSNSASQSFFWYRQDCRKEPKLLMSVYSSGNEDGRFTAQLNRASQYISLLIRDSKLSDSATYLCVVNTGRRALTFGSGTRLQVQP

SEQ ID NO: 131 - protein, 133 aa, Homo sapiens
MGFRLLCCVAFCLLGAGPVDSGVTQTPKHLITATGQRVTLRCSPRSGDLSVYWYQQSLDQGLQFLIQYYNGEERAKGNILERFSAQQFPDLHSELNLSSLELGDSALYFCASSVGGGAGNTIYFGEGSWLTVV

SEQ ID NO: 132 - protein, 131 aa, Homo sapiens
MAGIRALFMYLWLQLDWVSRGESVGLHLPTLSVQEGDNSIINCAYSNSASDYFIWYKQESGKGPQFIIDIRSNMDKRQGQRVTVLLNKTVKHLSLQIAATQPGDSAVYFCAGRTGFQKLVFGTGTRLLVSP

SEQ ID NO: 133 - protein, 133 aa, Homo sapiens
MGFRLLCCVAFCLLGAGPVDSGVTQTPKHLITATGQRVTLRCSPRSGDLSVYWYQQSLDQGLQFLIQYYNGEERAKGNILERFSAQQFPDLHSELNLSSLELGDSALYFCASSVGGGLYNEQFFGPGTRLTVL

SEQ ID NO: 134 - protein, 131 aa, Homo sapiens
METLLGVSLVILWLQLARVNSQQGEEDPQALSIQEGENATMNCSYKTSINNLQWYRQNSGRGLVHLILIRSNEREKHSGRLRVTLDTSKKSSSLLITASRAADTASYFCAVRYSSASKIIFGSGTRLSIRP

SEQ ID NO: 135 - protein, 133 aa, Homo sapiens
MGFRLLCCVAFCLLGAGPVDSGVTQTPKHLITATGQRVTLRCSPRSGDLSVYWYQQSLDQGLQFLIQYYNGEERAKGNILERFSAQQFPDLHSELNLSSLELGDSALYFCASSAGGGSNNEQFFGPGTRLTVL

SEQ ID NO: 136 - protein, 132 aa, Homo sapiens
MISLRVLLVILWLQLSWVWSQRKEVEQDPGPFNVPEGATVAFNCTYSNSASQSFFWYRQDCRKEPKLLMSVYSSGNEDGRFTAQLNRASQYISLLIRDSKLSDSATYLCVVKGGNNFNKFYFGSGTKLNVKP

SEQ ID NO: 137 - protein, 133 aa, Homo sapiens
MSIGLLCCVAFSLLWASPVNAGVTQTPKFQVLKTGQSMTLQCAQDMNHNSMYWYRQDPGMGLRLIYYSASEGTTDKGEVPNGYNVSRLNKREFSLRLESAAPSQTSVYFCASSHRVNSNQPQHFGDGTRLSIL

SEQ ID NO: 138 - protein, 128 aa, Homo sapiens
MKPTLISVLVIIFILRGTRAQRVTQPEKLLSVFKGAPVELKCNYSYSGSPELFWYVQYSRQRLQLLLRHISRESIKGFTADLNKGETSFHLKKPFAQEEDSAMYYCALANQAGTALIFGKGTTLSVSS

SEQ ID NO: 139 - protein, 132 aa, Homo sapiens
METLLGLLILWLQLQWVSSKQEVTQIPAALSVPEGENLVLNCSFTDSAIYNLQWFRQDPGKGLTSLLLIQSSQREQTSGRLNASLDKSSGRSTLYIAASQPGDSATYLCAVKRRAAGNKLTFGGGTRVLVKP

SEQ ID NO: 140 - protein, 133 aa, Homo sapiens
MGFRLLCCVAFCLLGAGPVDSGVTQTPKHLITATGQRVTLRCSPRSGDLSVYWYQQSLDQGLQFLIQYYNGEERAKGNILERFSAQQFPDLHSELNLSSLELGDSALYFCASSPGGGASSPLHFGNGTRLTVT

SEQ ID NO: 141 - protein, 130 aa, Homo sapiens
MISLRVLLVILWLQLSWVWSQRKEVEQDPGPFNVPEGATVAFNCTYSNSASQSFFWYRQDCRKEPKLLMSVYSSGNEDGRFTAQLNRASQYISLLIRDSKLSDSATYLCVVNKSWGKLQFGAGTQVVVTP

SEQ ID NO: 142 - protein, 132 aa, Homo sapiens
MGFRLLCCVAFCLLGAGPVDSGVTQTPKHLITATGQRVTLRCSPRSGDLSVYWYQQSLDQGLQFLIQYYNGEERAKGNILERFSAQQFPDLHSELNLSSLELGDSALYFCASSAGTSGNEQFFGPGTRLTVL

SEQ ID NO: 143 - protein, 129 aa, Homo sapiens
MWGVFLLYVSMKMGGTTGQNIDQPTEMTATEGAIVQINCTYQTSGFNGLFWYQQHAGEAPTFLSYNVLDGLEEKGRFSSFLSRSKGYSYLLLKELQMKDSASYLCAVRVWKAAGNKLTFGGGTRVLVKP

SEQ ID NO: 144 - protein, 131 aa, Homo sapiens
MLLLLLLLGPGSGLGAVVSQHPSWVICKSGTSVKIECRSLDFQATTMFWYRQFPKQSLMLMATSNEGSKATYEQGVEKDKFLINHASLTLSTLTVTSAHPEDSSFYICSARRLAGGGNEQFFGPGTRLTVL

SEQ ID NO: 145 - protein, 132 aa, Homo sapiens
MISLRVLLVILWLQLSWVWSQRKEVEQDPGPFNVPEGATVAFNCTYSNSASQSFFWYRQDCRKEPKLLMSVYSSGNEDGRFTAQLNRASQYISLLIRDSKLSDSATYLCVVNLGNYGQNFVFGPGTRLSVLP

SEQ ID NO: 146 - protein, 133 aa, Homo sapiens
MGFRLLCCVAFCLLGAGPVDSGVTQTPKHLITATGQRVTLRCSPRSGDLSVYWYQQSLDQGLQFLIQYYNGEERAKGNILERFSAQQFPDLHSELNLSSLELGDSALYFCASSVGGGLSNEQFFGPGTRLTVL

SEQ ID NO: 147 - protein, 130 aa, Homo sapiens
MKTFAGFSFLFLWLQLDCMSRGEDVEQSLFLSVREGDSSVINCTYTDSSSTYLYWYKQEPGAGLQLLTYIFSNMDMKQDQRLTVLLNKKDKHLSLRIADTQTGDSAIYFCAENHSSASKIIFRCGCGPAE

SEQ ID NO: 148 - protein, 133 aa, Homo sapiens
MGFRLLCCVAFCLLGAGPVDSGVTQTPKHLITATGQRVTLRCSPRSGDLSVYWYQQSLDQGLQFLIQYYNGEERAKGNILERFSAQQFPDLHSELNLSSLELGDSALYFCASSVGSGRNYEQYFGPGTRLTVT

SEQ ID NO: 149 - DNA, 388 bp, Homo sapiens
  source 1..388: mol_type = other DNA
atggtcctgaaattctccgtgtccattctttggattcagttggcatgggtgagcacccagctgctggagcagagccctcagtttctaagcatccaagagggagaaaatctcactgtgtactgcaactcctcaagtgttttttccagcttacaatggtacagacaggagcctggggaaggtcctgtcctcctggtgacagtagttacgggtggagaagtgaagaagctgaagagactaacctttcagtttggtgatgcaagaaaggacagttctctccacatcactgcagcccagcctggtgatacaggcctctacctctgtgcaggccggtacagcagtgcttccaagataatctttggatcagggaccagactcagcatccggccaa

SEQ ID NO: 150 - DNA, 399 bp, Homo sapiens
  source 1..399: mol_type = other DNA
atgggcttcaggctcctctgctgtgtggccttttgtctcctgggagcaggcccagtggattctggagtcacacaaaccccaaagcacctgatcacagcaactggacagcgagtgacgctgagatgctcccctaggtctggagacctctctgtgtactggtaccaacagagcctggaccagggcctccagttcctcattcagtattataatggagaagagagagcaaaaggaaacattcttgaacgattctccgcacaacagttccctgacttgcactctgaactaaacctgagctctctggagctgggggactcagctttgtatttctgtgccagcagcgtaggcgggggggcacccaatgagcagttcttcgggccagggacacggctcaccgtgcta

SEQ ID NO: 151 - DNA, 385 bp, Homo sapiens
  source 1..385: mol_type = other DNA
atggagaccctcttgggcctgcttatcctttggctgcagctgcaatgggtgagcagcaaacaggaggtgacacagattcctgcagctctgagtgtcccagaaggagaaaacttggttctcaactgcagtttcactgatagcgctatttacaacctccagtggtttaggcaggaccctgggaaaggtctcacatctctgttgcttattcagtcaagtcagagagagcaaacaagtggaagacttaatgcctcgctggataaatcatcaggacgtagtactttatacattgcagcttctcagcctggtgactcagccacctacctctgtgctgttaccaggagagcacttacttttgggagtggaacaagactccaagtgcaaccaa

SEQ ID NO: 152 - DNA, 405 bp, Homo sapiens
  source 1..405: mol_type = other DNA
atgggctccaggctgctctgttgggtgctgctttgtctcctgggagcaggcccagtaaaggctggagtcactcaaactccaagatatctgatcaaaacgagaggacagcaagtgacactgagctgctcccctatctctgggcataggagtgtatcctggtaccaacagaccccaggacagggccttcagttcctctttgaatacttcagtgagacacagagaaacaaaggaaacttccctggtcgattctcagggcgccagttctctaactctcgctctgagatgaatgtgagcaccttggagctgggggactcggccctttatctttgcgccagcagcgtaactagcgggagaacacacacagatacgcagtattttggcccaggcacccggctgacagtgctc

SEQ ID NO: 153 - DNA, 394 bp, Homo sapiens
  source 1..394: mol_type = other DNA
atgatgatatccttgagagttttactggtgatcctgtggcttcagttaagctgggtttggagccaacggaaggaggtggagcaggatcctggacccttcaatgttccagagggagccactgtcgctttcaactgtacttacagcaacagtgcttctcagtctttcttctggtacagacaggattgcaggaaagaacctaagttgctgatgtccgtatactccagtggtaatgaagatggaaggtttacagcacagctcaatagagccagccagtatatttccctgctcatcagagactccaagctcagtgattcagccacctacctctgtaagatttctggtggctacaataagctgatttttggagcagggaccaggctggctgtacacccat

SEQ ID NO: 154 - DNA, 399 bp, Homo sapiens
  source 1..399: mol_type = other DNA
atgggcttcaggctcctctgctgtgtggccttttgtctcctgggagcaggcccagtggattctggagtcacacaaaccccaaagcacctgatcacagcaactggacagcgagtgacgctgagatgctcccctaggtctggagacctctctgtgtactggtaccaacagagcctggaccagggcctccagttcctcattcagtattataatggagaagagagagcaaaaggaaacattcttgaacgattctccgcacaacagttccctgacttgcactctgaactaaacctgagctctctggagctgggggactcagctttgtatttctgtgccagcagcgtaggtgggggtttagggactgaagctttctttggacaaggcaccagactcacagttgta

SEQ ID NO: 155 - DNA, 382 bp, Homo sapiens
  source 1..382: mol_type = other DNA
atgaggcaagtggcgagagtgatcgtgttcctgaccctgagtactttgagccttgctaagaccacccagcccatctccatggactcatatgaaggacaagaagtgaacataacctgtagccacaacaacattgctacaaatgattatatcacgtggtaccaacagtttcccagccaaggaccacgatttattattcaaggatacaagacaaaagttacaaacgaagtggcctccctgtttatccctgccgacagaaagtccagcactctgagcctgccccgggtttccctgagcgacactgctgtgtactactgcctcgtgggacattcaggaaacacacctcttgtctttggaaagggcacaagactttctgtgattgcaa

SEQ ID NO: 156 - DNA, 399 bp, Homo sapiens
  source 1..399: mol_type = other DNA
atgggcttcaggctcctctgctgtgtggccttttgtctcctgggagcaggcccagtggattctggagtcacacaaaccccaaagcacctgatcacagcaactggacagcgagtgacgctgagatgctcccctaggtctggagacctctctgtgtactggtaccaacagagcctggaccagggcctccagttcctcattcagtattataatggagaagagagagcaaaaggaaacattcttgaacgattctccgcacaacagttccctgacttgcactctgaactaaacctgagctctctggagctgggggactcagctttgtatttctgtgccagcagcgtaggagggggagctggaaacaccatatattttggagagggaagttggctcactgttgta

SEQ ID NO: 157 - DNA, 390 bp, Homo sapiens
  source 1..390: mol_type = other DNA
atgatatccttgagagttttactggtgatcctgtggcttcagttaagctgggtttggagccaacggaaggaggtggagcaggatcctggacccttcaatgttccagagggagccactgtcgctttcaactgtacttacagcaacagtgcttctcagtctttcttctggtacagacaggattgcaggaaagaacctaagttgctgatgtccgtatactccagtggtaatgaagatggaaggtttacagcacagctcaatagagccagccagtatatttccctgctcatcagagactccaagctcagtgattcagccacctacctctgtgtggtgaacacgggcaggagagcacttacttttgggagtggaacaagactccaagtgcaacca

SEQ ID NO: 158 - DNA, 399 bp, Homo sapiens; identical to SEQ ID NO: 156
  source 1..399: mol_type = other DNA

SEQ ID NO: 159 - DNA, 393 bp, Homo sapiens
  source 1..393: mol_type = other DNA
atggcaggcattcgagctttatttatgtacttgtggctgcagctggactgggtgagcagaggagagagtgtggggctgcatcttcctaccctgagtgtccaggagggtgacaactctattatcaactgtgcttattcaaacagcgcctcagactacttcatttggtacaagcaagaatctggaaaaggtcctcaattcattatagacattcgttcaaatatggacaaaaggcaaggccaaagagtcaccgttttattgaataagacagtgaaacatctctctctgcaaattgcagctactcaacctggagactcagctgtctacttttgtgcagggcgaacaggctttcagaaacttgtatttggaactggcacccgacttctggtcagtcca

SEQ ID NO: 160 - DNA, 399 bp, Homo sapiens
  source 1..399: mol_type = other DNA
atgggcttcaggctcctctgctgtgtggccttttgtctcctgggagcaggcccagtggattctggagtcacacaaaccccaaagcacctgatcacagcaactggacagcgagtgacgctgagatgctcccctaggtctggagacctctctgtgtactggtaccaacagagcctggaccagggcctccagttcctcattcagtattataatggagaagagagagcaaaaggaaacattcttgaacgattctccgcacaacagttccctgacttgcactctgaactaaacctgagctctctggagctgggggactcagctttgtatttctgtgccagcagcgtaggaggggggctctacaatgagcagttcttcgggccagggacacggctcaccgtgcta

SEQ ID NO: 161 - DNA, 394 bp, Homo sapiens
  source 1..394: mol_type = other DNA
atggaaactctcctgggagtgtctttggtgattctatggcttcaactggctagggtgaacagtcaacagggagaagaggatcctcaggccttgagcatccaggagggtgaaaatgccaccatgaactgcagttacaaaactagtataaacaatttacagtggtatagacaaaattcaggtagaggccttgtccacctaattttaatacgttcaaatgaaagagagaaacacagtggaagattaagagtcacgcttgacacttccaagaaaagcagttccttgttgatcacggcttcccgggcagcagacactgcttcttacttctgtgctgtgaggtacagcagtgcttccaagataatctttggatcagggaccagactcagcatccggccaa

SEQ ID NO: 162 - DNA, 399 bp, Homo sapiens
  source 1..399: mol_type = other DNA
atgggcttcaggctcctctgctgtgtggccttttgtctcctgggagcaggcccagtggattctggagtcacacaaaccccaaagcacctgatcacagcaactggacagcgagtgacgctgagatgctcccctaggtctggagacctctctgtgtactggtaccaacagagcctggaccagggcctccagttcctcattcagtattataatggagaagagagagcaaaaggaaacattcttgaacgattctccgcacaacagttccctgacttgcactctgaactaaacctgagctctctggagctgggggactcagctttgtatttctgtgccagcagcgcaggagggggtagtaacaatgagcagttcttcgggccagggacacggctcaccgtgcta

SEQ ID NO: 163 - DNA, 397 bp, Homo sapiens
  source 1..397: mol_type = other DNA
atgatatccttgagagttttactggtgatcctgtggcttcagttaagctgggtttggagccaacggaaggaggtggagcaggatcctggacccttcaatgttccagagggagccactgtcgctttcaactgtacttacagcaacagtgcttctcagtctttcttctggtacagacaggattgcaggaaagaacctaagttgctgatgtccgtatactccagtggtaatgaagatggaaggtttacagcacagctcaatagagccagccagtatatttccctgctcatcagagactccaagctcagtgattcagccacctacctctgtgtggtgaaaggtgggaacaacttcaacaaattttactttggatctgggaccaaactcaatgtaaaaccaa

SEQ ID NO: 164 - DNA, 399 bp, Homo sapiens
  source 1..399: mol_type = other DNA
atgagcatcgggctcctgtgctgtgtggccttttctctcctgtgggcaagtccagtgaatgctggtgtcactcagaccccaaaattccaggtcctgaagacaggacagagcatgacactgcagtgtgcccaggatatgaaccataactccatgtactggtatcgacaagacccaggcatgggactgaggctgatttattactcagcttctgagggtaccactgacaaaggagaagtccccaatggctacaatgtctccagattaaacaaacgggagttctcgctcaggctggagtcggctgctccctcccagacatctgtgtacttctgtgccagcagccacagggttaatagcaatcagccccagcattttggtgatgggactcgactctccatccta

SEQ ID NO: 165 - DNA, 385 bp, Homo sapiens
  source 1..385: mol_type = other DNA
atgaagcccaccctcatctcagtgcttgtgataatatttatactcagaggaacaagagcccagagagtgactcagcccgagaagctcctctctgtctttaaaggggccccagtggagctgaagtgcaactattcctattctgggagtcctgaactcttctggtatgtccagtactccagacaacgcctccagttactcttgagacacatctctagagagagcatcaaaggcttcactgctgaccttaacaaaggcgagacatctttccacctgaagaaaccatttgctcaagaggaagactcagccatgtattactgtgctcttgccaaccaggcaggaactgctctgatctttgggaagggaaccaccttatcagtgagttcca

SEQ ID NO: 166 - DNA, 399 bp, Homo sapiens
  source 1..399: mol_type = other DNA
atgggcttcaggctcctctgctgtgtggccttttgtctcctgggagcaggcccagtggattctggagtcacacaaaccccaaagcacctgatcacagcaactggacagcgagtgacgctgagatgctcccctaggtctggagacctctctgtgtactggtaccaacagagcctggaccagggcctccagttcctcattcagtattataatggagaagagagagcaaaaggaaacattcttgaacgattctccgcacaacagttccctgacttgcactctgaactaaacctgagctctctggagctgggggactcagctttgtatttctgtgccagcagcccgggtggaggggcgagttcacccctccactttgggaatgggaccaggctcactgtgaca

SEQ ID NO: 167 - DNA, 397 bp, Homo sapiens
  source 1..397: mol_type = other DNA
atggagaccctcttgggcctgcttatcctttggctgcagctgcaatgggtgagcagcaaacaggaggtgacacagattcctgcagctctgagtgtcccagaaggagaaaacttggttctcaactgcagtttcactgatagcgctatttacaacctccagtggtttaggcaggaccctgggaaaggtctcacatctctgttgcttattcagtcaagtcagagagagcaaacaagtggaagacttaatgcctcgctggataaatcatcaggacgtagtactttatacattgcagcttctcagcctggtgactcagccacctacctctgtgctgtgaaacgacgagctgcaggcaacaagctaacttttggaggaggaaccagggtgctagttaaaccaa

SEQ ID NO: 168 - DNA, 399 bp, Homo sapiens; identical to SEQ ID NO: 166
  source 1..399: mol_type = other DNA

SEQ ID NO: 169 - DNA, 391 bp, Homo sapiens
  source 1..391: mol_type = other DNA
atgatatccttgagagttttactggtgatcctgtggcttcagttaagctgggtttggagccaacggaaggaggtggagcaggatcctggacccttcaatgttccagagggagccactgtcgctttcaactgtacttacagcaacagtgcttctcagtctttcttctggtacagacaggattgcaggaaagaacctaagttgctgatgtccgtatactccagtggtaatgaagatggaaggtttacagcacagctcaatagagccagccagtatatttccctgctcatcagagactccaagctcagtgattcagccacctacctctgtgtggtgaacaagagctgggggaaattgcagtttggagcagggacccaggttgtggtcaccccag

SEQ ID NO: 170 - protein, 396 aa, Homo sapiens
ATGGGCTTCAGGCTCCTCTGCTGTGTGGCCTTTTGTCTCCTGGGAGCAGGCCCAGTGGATTCTGGAGTCACACAAACCCCAAAGCACCTGATCACAGCAACTGGACAGCGAGTGACGCTGAGATGCTCCCCTAGGTCTGGAGACCTCTCTGTGTACTGGTACCAACAGAGCCTGGACCAGGGCCTCCAGTTCCTCATTCAGTATTATAATGGAGAAGAGAGAGCAAAAGGAAACATTCTTGAACGATTCTCCGCACAACAGTTCCCTGACTTGCACTCTGAACTAAACCTGAGCTCTCTGGAGCTGGGGGACTCAGCTTTGTATTTCTGTGCCAGCAGCGCCGGGACTAGCGGAAATGAGCAGTTCTTCGGGCCAGGGACACGGCTCACCGTGCTA

SEQ ID NO: 171 - DNA, 388 bp, Homo sapiens
  source 1..388: mol_type = other DNA
atgtggggagttttccttctttatgtttccatgaagatgggaggcactacaggacaaaacattgaccagcccactgagatgacagctacggaaggtgccattgtccagatcaactgcacgtaccagacatctgggttcaacgggctgttctggtaccagcaacatgctggcgaagcacccacatttctgtcttacaatgttctggatggtttggaggagaaaggtcgtttttcttcattccttagtcggtctaaagggtacagttacctccttttgaaggagctccagatgaaagactctgcctcttacctctgtgctgtgagagtgtggaaagctgcaggcaacaagctaacttttggaggaggaaccagggtgctagttaaaccaa

SEQ ID NO: 172 - DNA, 393 bp, Homo sapiens
  source 1..393: mol_type = other DNA
atgctgctgcttctgctgcttctggggccaggctccgggcttggtgctgtcgtctctcaacatccgagctgggttatctgtaagagtggaacctctgtgaagatcgagtgccgttccctggactttcaggccacaactatgttttggtatcgtcagttcccgaaacagagtctcatgctgatggcaacttccaatgagggctccaaggccacatacgagcaaggcgtcgagaaggacaagtttctcatcaaccatgcaagcctgaccttgtccactctgacagtgaccagtgcccatcctgaagacagcagcttctacatctgcagtgctagaaggctagcgggaggagggaatgagcagttcttcgggccagggacacggctcaccgtgcta

SEQ ID NO: 173 - DNA, 397 bp, Homo sapiens
  source 1..397: mol_type = other DNA
atgatatccttgagagttttactggtgatcctgtggcttcagttaagctgggtttggagccaacggaaggaggtggagcaggatcctggacccttcaatgttccagagggagccactgtcgctttcaactgtacttacagcaacagtgcttctcagtctttcttctggtacagacaggattgcaggaaagaacctaagttgctgatgtccgtatactccagtggtaatgaagatggaaggtttacagcacagctcaatagagccagccagtatatttccctgctcatcagagactccaagctcagtgattcagccacctacctctgtgtggtgaacctcgggaactatggtcagaattttgtctttggtcccggaaccagattgtccgtgctgccct

SEQ ID NO: 174 - DNA, 399 bp, Homo sapiens
  source 1..399: mol_type = other DNA
atgggcttcaggctcctctgctgtgtggccttttgtctcctgggagcaggcccagtggattctggagtcacacaaaccccaaagcacctgatcacagcaactggacagcgagtgacgctgagatgctcccctaggtctggagacctctctgtgtactggtaccaacagagcctggaccagggcctccagttcctcattcagtattataatggagaagagagagcaaaaggaaacattcttgaacgattctccgcacaacagttccctgacttgcactctgaactaaacctgagctctctggagctgggggactcagctttgtatttctgtgccagcagcgtaggggggggcctaagcaatgagcagttcttcgggccagggacacggctcaccgtgcta

SEQ ID NO: 175 - DNA, 390 bp, Homo sapiens
  source 1..390: mol_type = other DNA
atgaagacatttgctggattttcgttcctgtttttgtggctgcagctggactgtatgagtagaggagaggatgtggagcagagtcttttcctgagtgtccgagagggagacagctccgttataaactgcacttacacagacagctcctccacctacttatactggtataagcaagaacctggagcaggtctccagttgctgacgtatattttttcaaatatggacatgaaacaagaccaaagactcactgttctattgaataaaaaggataaacatctgtctctgcgcattgcagacacccagactggggactcagctatctacttctgtgcagagaaccacagcagtgcttccaagataatctttcgctgcggctgtggtccagctgaa

SEQ ID NO: 176 - DNA, 399 bp, Homo sapiens
  source 1..399: mol_type = other DNA
atgggcttcaggctcctctgctgtgtggccttttgtctcctgggagcaggcccagtggattctggagtcacacaaaccccaaagcacctgatcacagcaactggacagcgagtgacgctgagatgctcccctaggtctggagacctctctgtgtactggtaccaacagagcctggaccagggcctccagttcctcattcagtattataatggagaagagagagcaaaaggaaacattcttgaacgattctccgcacaacagttccctgacttgcactctgaactaaacctgagctctctggagctgggggactcagctttgtatttctgtgccagcagcgtagggtcgggacgaaattacgagcagtacttcgggccgggcaccaggctcacggtcaca

SEQ ID NO: 177 - protein, 130 aa, Homo sapiens
MALQSTLGAVWLGLLLNSLWKVAESKDQVFQPSTVASSEGAVVEIFCNHSVSNAYNFFWYLHFPGCAPRLLVKGSKPSQQGRYNMTYERFSSSLLILQVREADAAVYYCAVNQAGTALIFGKGTTLSVSS

SEQ ID NO: 178 - protein, 137 aa, Homo sapiens
MGCRLLCCAVLCLLGAVPIDTEVTQTPKHLVMGMTNKKSLKCEQHMGHRAMYWYKQKAKKPPELMFVYSYEKLSINESVPSRFSPECPNSSLLNLHLHALQPEDSALYLCASSQERTSGRSADTQYFGPGTRLTVLE

SEQ ID NO: 179 - protein, 135 aa, Homo sapiens
MLLLLIPVLGMIFALRDARAQSVSQHNHHVILSEAASLELGCNYSYGGTVNLFWYVQYPGQHLQLLLKYFSGDPLVKGIKGFEAEFIKSKFSFNLRKPSVQWSDTAEYFCAVRHGGTGTASKLTFGTGTRLQVTL

SEQ ID NO: 180 - protein, 139 aa, Homo sapiens
MLLLLLLLGPGISLLLPGSLAGSGLGAVVSQHPSWVICKSGTSVKIECRSLDFQATTMFWYRQFPKQSLMLMATSNEGSKATYEQGVEKDKFLINHASLTLSTLTVTSAHPEDSSFYICSARALGGYTFGSGTRLTVVE

SEQ ID NO: 181 - protein, 132 aa, Homo sapiens
MMKSLRVLLVILWLQLSWVWSQQKEVEQDPGPLSVPEGAIVSLNCTYSNSAFQYFMWYRQYSRKGPELLMYTYSSGNKEDGRFTAQVDKSSKYISLFIRDSQPSDSATYLCAMSGHFNKFYFGSGTKLNVKP

SEQ ID NO: 182 - protein, 131 aa, Homo sapiens
MGSRLLCWVLLCLLGAGPVKAGVTQTPRYLIKTRGQQVTLSCSPISGHRSVSWYQQTPGQGLQFLFEYFSETQRNKGNFPGRFSGRQFSNSRSEMNVSTLELGDSALYLCASSLRAGELFFGEGSRLTVLE

SEQ ID NO: 183 - protein, 133 aa, Homo sapiens
MEKMLECAFIVLWLQLGWLSGEDQVTQSPEALRLQEGESSSLNCSYTVSGLRGLFWYRQDPGKGPEFLFTLYSAGEEKEKERLKATLTKKESFLHITAPKPEDSATYLCAASNSGGSNYKLTFGKGTLLTVNP

SEQ ID NO: 184 - protein, 132 aa, Homo sapiens
MGFRLLCCVAFCLLGAGPVDSGVTQTPKHLITATGQRVTLRCSPRSGDLSVYWYQQSLDQGLQFLIQYYNGEERAKGNILERFSAQQFPDLHSELNLSSLELGDSALYFCASSVDGKGTQYFGPGTRLLVLE

SEQ ID NO: 185 - DNA, 391 bp, Homo sapiens
  source 1..391: mol_type = other DNA
atggctttgcagagcactctgggggcggtgtggctagggcttctcctcaactctctctggaaggttgcagaaagcaaggaccaagtgtttcagccttccacagtggcatcttcagagggagctgtggtggaaatcttctgtaatcactctgtgtccaatgcttacaacttcttctggtaccttcacttcccgggatgtgcaccaagactccttgttaaaggctcaaagccttctcagcagggacgatacaacatgacctatgaacggttctcttcatcgctgctcatcctccaggtgcgggaggcagatgctgctgtttactactgtgctgttaaccaggcaggaactgctctgatctttgggaagggaaccaccttatcagtgagttcca

SEQ ID NO: 186 - DNA, 408 bp, Homo sapiens
  source 1..408: mol_type = other DNA
atgggctgcaggctgctctgctgtgcggttctctgtctcctgggagcagttcccatagacactgaagttacccagacaccaaaacacctggtcatgggaatgacaaataagaagtctttgaaatgtgaacaacatatggggcacagggctatgtattggtacaagcagaaagctaagaagccaccggagctcatgtttgtctacagctatgagaaactctctataaatgaaagtgtgccaagtcgcttctcacctgaatgccccaacagctctctcttaaaccttcacctacacgccctgcagccagaagactcagccctgtatctctgcgccagcagccaagagcggactagcgggaggtcggcagatacgcagtattttggcccaggcacccggctgacagtgctc

SEQ ID NO: 187 - DNA, 406 bp, Homo sapiens
  source 1..406: mol_type = other DNA
atgctcctgttgctcataccagtgctggggatgatttttgccctgagagatgccagagcccagtctgtgagccagcataaccaccacgtaattctctctgaagcagcctcactggagttgggatgcaactattcctatggtggaactgttaatctcttctggtatgtccagtaccctggtcaacaccttcagcttctcctcaagtacttttcaggggatccactggttaaaggcatcaagggctttgaggctgaatttataaagagtaaattctcctttaatctgaggaaaccctctgtgcagtggagtgacacagctgagtacttctgtgccgtgaggcacggcggtaccggcactgccagtaaactcacctttgggactggaacaagacttcaggtcacgctcg

SEQ ID NO: 188 - DNA, 414 bp, Homo sapiens
  source 1..414: mol_type = other DNA
atgctgctgcttctgctgcttctggggccaggtataagcctccttctacctgggagcttggcaggctccgggcttggtgctgtcgtctctcaacatccgagctgggttatctgtaagagtggaacctctgtgaagatcgagtgccgttccctggactttcaggccacaactatgttttggtatcgtcagttcccgaaacagagtctcatgctgatggcaacttccaatgagggctccaaggccacatacgagcaaggcgtcgagaaggacaagtttctcatcaaccatgcaagcctgaccttgtccactctgacagtgaccagtgcccatcctgaagacagcagcttctacatctgcagtgctagagctttaggaggctacaccttcggttcggggaccaggttaaccgttgta

SEQ ID NO: 189 - DNA, 397 bp, Homo sapiens
  source 1..397: mol_type = other DNA
atgatgaaatccttgagagttttactggtgatcctgtggcttcagttaagctgggtttggagccaacagaaggaggtggagcaggatcctggaccactcagtgttccagagggagccattgtttctctcaactgcacttacagcaacagtgcttttcaatacttcatgtggtacagacagtattccagaaaaggccctgagttgctgatgtacacatactccagtggtaacaaagaagatggaaggtttacagcacaggtcgataaatccagcaagtatatctccttgttcatcagagactcacagcccagtgattcagccacctacctctgtgcaatgagcggtcacttcaacaaattttactttggatctgggaccaaactcaatgtaaaaccaa

SEQ ID NO: 190 - DNA, 390 bp, Homo sapiens
  source 1..390: mol_type = other DNA
atgggctccaggctgctctgttgggtgctgctttgtctcctgggagcaggcccagtaaaggctggagtcactcaaactccaagatatctgatcaaaacgagaggacagcaagtgacactgagctgctcccctatctctgggcataggagtgtatcctggtaccaacagaccccaggacagggccttcagttcctctttgaatacttcagtgagacacagagaaacaaaggaaacttccctggtcgattctcagggcgccagttctctaactctcgctctgagatgaatgtgagcaccttggagctgggggactcggccctttatctttgcgccagcagcttgcgggccggggagctgttttttggagaaggctctaggctgaccgtactg

SEQ ID NO: 191 - DNA, 400 bp, Homo sapiens
  source 1..400: mol_type = other DNA
atggagaaaatgttggagtgtgcattcatagtcttgtggcttcagcttggctggttgagtggagaagaccaggtgacgcagagtcccgaggccctgagactccaggagggagagagtagcagtctcaactgcagttacacagtcagcggtttaagagggctgttctggtataggcaagatcctgggaaaggccctgaattcctcttcaccctgtattcagctggggaagaaaaggagaaagaaaggctaaaagccacattaacaaagaaggaaagctttctgcacatcacagcccctaaacctgaagactcagccacttatctctgtgctgcctccaatagtggaggtagcaactataaactgacatttggaaaaggaactctcttaaccgtgaatccaa

SEQ ID NO: 192 - DNA, 393 bp, Homo sapiens
  source 1..393: mol_type = other DNA
atgggcttcaggctcctctgctgtgtggccttttgtctcctgggagcaggcccagtggattctggagtcacacaaaccccaaagcacctgatcacagcaactggacagcgagtgacgctgagatgctcccctaggtctggagacctctctgtgtactggtaccaacagagcctggaccagggcctccagttcctcattcagtattataatggagaagagagagcaaaaggaaacattcttgaacgattctccgcacaacagttccctgacttgcactctgaactaaacctgagctctctggagctgggggactcagctttgtatttctgtgccagcagcgtagacgggaaggggacccagtacttcgggccaggcacgcggctcctggtgctc

SEQ ID NO: 193 - protein, 136 aa, Homo sapiens
MACPGFLWALVISTCLEFSMAQTVTQSQPEMSVQEAETVTLSCTYDTSESDYYLFWYKQPPSRQMILVIRQEAYKQQNATENRFSVNFQKAAKSFSLKISDSQLGDAAMYFCAYRIPGAGSYQLTFGKGTKLSVIP

SEQ ID NO: 194 - protein, 136 aa, Homo sapiens
MGTRLLCWVVLGFLGTDHTGAGVSQSPRYKVAKRGQDVALRCDPISGHVSLFWYQQALGQGPEFLTYFQNEAQLDKSGLPSDRFFAERPEGSVSTLKIQRTQQEDSAVYLCASSPGLAGGAQETQYFGPGTRLLVL

SEQ ID NO: 195 - protein, 131 aa, Homo sapiens
METLLGVSLVILWLQLARVNSQQGEEDPQALSIQEGENATMNCSYKTSINNLQWYRQNSGRGLVHLILIRSNEREKHSGRLRVTLDTSKKSSSLLITASRAADTASYFCATDTGGAQKLVFGQGTRLTINP

SEQ ID NO: 196 - protein, 132 aa, Homo sapiens
MDSWTLCCVSLCILVAKHTDAGVIQSPRHEVTEMGQEVTLRCKPISGHDYLFWYRQTMMRGLELLIYFNNNVPIDDSGMPEDRFSAKMPNASFSTLKIQPSEPRDSAVYFCASSPDRGETQYFGPGTRLLVL

SEQ ID NO: 197 - protein, 129 aa, Homo sapiens
MWGVFLLYVSMKMGGTTGQNIDQPTEMTATEGAIVQINCTYQTSGFNGLFWYQQHAGEAPTFLSYNVLDGLEEKGRFSSFLSRSKGYSYLLLKELQMKDSASYLCAVRALREAGTALIFGKGTTLSVSS

SEQ ID NO: 198 - protein, 130 aa, Homo sapiens
MDTWLVCWAIFSLLKAGLTEPEVTQTPSHQVTQMGQEVILRCVPISNHLYFYWYRQILGQKVEFLVSFYNNEISEKSEIFDDQFSVERPDGSNFTLKIRSTKLEDSAMYFCASSQNREAFFGQGTRLTVV

SEQ ID NO: 199 - protein, 126 aa, Homo sapiens
MISLRVLLVILWLQLSWVWSQRKEVEQDPGPFNVPEGATVAFNCTYSNSASQSFFWYRQDCRKEPKLLMSVYSSGNEDGRFTAQLNRASQYISLLIRDSKLSDSATYLCVVSARVFGSGTRLSIRP

SEQ ID NO: 200 - protein, 137 aa, Homo sapiens
MMKSLRVLLVILWLQLSWVWSQQKEVEQDPGPLSVPEGAIVSLNCTYSNSAFQYFMWYRQYSRKGPELLMYTYSSGNKEDGRFTAQVDKSSKYISLFIRDSQPSDSATYLCAMSVRGSGAGSYQLTFGKGTKLSVIP

SEQ ID NO: 201 - protein, 134 aa, Homo sapiens
MGTSLLCWMALCLLGADHADTGVSQDPRHKITKRGQNVTFRCDPISEHNRLYWYRQTLGQGPEFLTYFQNEAQLEKSRLLSDRFSAERPKGSFSTLEIQRTEQGDSAMYLCASSPLAGVRYEQYFGPGTRLTVT

SEQ ID NO: 202 - protein, 135 aa, Homo sapiens
MSLSSLLKVVTASLWLGPGIAQKITQTQPGMFVQEKEAVTLDCTYDTSDPSYGLFWYKQPSSGEMIFLIYQGSYDQQNATEGRYSLNFQKARKSANLVISASQLGDSAMYFCAMRDRNTGNQFYFGTGTSLTVIP

SEQ ID NO: 203 - protein, 131 aa, Homo sapiens
MGFRLLCCVAFCLLGAGPVDSGVTQTPKHLITATGQRVTLRCSPRSGDLSVYWYQQSLDQGLQFLIQYYNGEERAKGNILERFSAQQFPDLHSELNLSSLELGDSALYFCASSVEVYNEQFFGPGTRLTVL

SEQ ID NO: 204 - DNA, 409 bp, Homo sapiens
  source 1..409: mol_type = other DNA
atggcatgccctggcttcctgtgggcacttgtgatctccacctgtcttgaatttagcatggctcagacagtcactcagtctcaaccagagatgtctgtgcaggaggcagagaccgtgaccctgagctgcacatatgacaccagtgagagtgattattatttattctggtacaagcagcctcccagcaggcagatgattctcgttattcgccaagaagcttataagcaacagaatgcaacagagaatcgtttctctgtgaacttccagaaagcagccaaatccttcagtctcaagatctcagactcacagctgggggatgccgcgatgtatttctgtgcttataggatcccgggtgctgggagttaccaactcactttcgggaaggggaccaaactctcggtcataccaa

SEQ ID NO: 205 - DNA, 408 bp, Homo sapiens
  source 1..408: mol_type = other DNA
atgggcaccaggctcctctgctgggtggtcctgggtttcctagggacagatcacacaggtgctggagtctcccagtcccctaggtacaaagtcgcaaagagaggacaggatgtagctctcaggtgtgatccaatttcgggtcatgtatcccttttttggtaccaacaggccctggggcaggggccagagtttctgacttatttccagaatgaagctcaactagacaaatcggggctgcccagtgatcgcttctttgcagaaaggcctgagggatccgtctccactctgaagatccagcgcacacagcaggaggactccgccgtgtatctctgtgccagcagcccgggtttagcgggaggggcccaagagacccagtacttcgggccaggcacgcggctcctggtgctc

SEQ ID NO: 206 - DNA, 394 bp, Homo sapiens
  source 1..394: mol_type = other DNA
atggaaactctcctgggagtgtctttggtgattctatggcttcaactggctagggtgaacagtcaacagggagaagaggatcctcaggccttgagcatccaggagggtgaaaatgccaccatgaactgcagttacaaaactagtataaacaatttacagtggtatagacaaaattcaggtagaggccttgtccacctaattttaatacgttcaaatgaaagagagaaacacagtggaagattaagagtcacgcttgacacttccaagaaaagcagttccttgttgatcacggcttcccgggcagcagacactgcttcttacttctgtgctacggacacggggggagcccagaagctggtatttggccaaggaaccaggctgactatcaacccaa

SEQ ID NO: 207 - DNA, 396 bp, Homo sapiens
  source 1..396: mol_type = other DNA
atggactcctggaccctctgctgtgtgtccctttgcatcctggtagcaaagcacacagatgctggagttatccagtcaccccggcacgaggtgacagagatgggacaagaagtgactctgagatgtaaaccaatttcaggacacgactaccttttctggtacagacagaccatgatgcggggactggagttgctcatttactttaacaacaacgttccgatagatgattcagggatgcccgaggatcgattctcagctaagatgcctaatgcatcattctccactctgaagatccagccctcagaacccagggactcagctgtgtacttctgtgccagcagcccggacaggggggagacccagtacttcgggccaggcacgcggctcctggtgctc

SEQ ID NO: 208 - DNA, 388 bp, Homo sapiens
  source 1..388: mol_type = other DNA
atgtggggagttttccttctttatgtttccatgaagatgggaggcactacaggacaaaacattgaccagcccactgagatgacagctacggaaggtgccattgtccagatcaactgcacgtaccagacatctgggttcaacgggctgttctggtaccagcaacatgctggcgaagcacccacatttctgtcttacaatgttctggatggtttggaggagaaaggtcgtttttcttcattccttagtcggtctaaagggtacagttacctccttttgaaggagctccagatgaaagactctgcctcttacctctgtgctgtgagagccctccgggaggcaggaactgctctgatctttgggaagggaaccaccttatcagtgagttcca

SEQ ID NO: 209 - DNA, 390 bp, Homo sapiens
  source 1..390: mol_type = other DNA
atggatacctggctcgtatgctgggcaatttttagtctcttgaaagcaggactcacagaacctgaagtcacccagactcccagccatcaggtcacacagatgggacaggaagtgatcttgcgctgtgtccccatctctaatcacttatacttctattggtacagacaaatcttggggcagaaagtcgagtttctggtttccttttataataatgaaatctcagagaagtctgaaatattcgatgatcaattctcagttgaaaggcctgatggatcaaatttcactctgaagatccggtccacaaagctggaggactcagccatgtacttctgtgccagcagtcaaaatcgggaagctttctttggacaaggcaccagactcacagttgta

SEQ ID NO: 210 - DNA, 379 bp, Homo sapiens
  source 1..379: mol_type = other DNA
atgatatccttgagagttttactggtgatcctgtggcttcagttaagctgggtttggagccaacggaaggaggtggagcaggatcctggacccttcaatgttccagagggagccactgtcgctttcaactgtacttacagcaacagtgcttctcagtctttcttctggtacagacaggattgcaggaaagaacctaagttgctgatgtccgtatactccagtggtaatgaagatggaaggtttacagcacagctcaatagagccagccagtatatttccctgctcatcagagactccaagctcagtgattcagccacctacctctgtgtggtgagcgcccgggtctttggatcagggaccagactcagcatccggccaa

SEQ ID NO: 211 - DNA, 412 bp, Homo sapiens
  source 1..412: mol_type = other DNA
atgatgaaatccttgagagttttactggtgatcctgtggcttcagttaagctgggtttggagccaacagaaggaggtggagcaggatcctggaccactcagtgttccagagggagccattgtttctctcaactgcacttacagcaacagtgcttttcaatacttcatgtggtacagacagtattccagaaaaggccctgagttgctgatgtacacatactccagtggtaacaaagaagatggaaggtttacagcacaggtcgataaatccagcaagtatatctccttgttcatcagagactcacagcccagtgattcagccacctacctctgtgcaatgagcgtcagaggctctggggctgggagttaccaactcactttcgggaaggggaccaaactctcggtcataccaa

SEQ ID NO: 212 - DNA, 402 bp, Homo sapiens
  source 1..402: mol_type = other DNA
atgggcaccagcctcctctgctggatggccctgtgtctcctgggggcagatcacgcagatactggagtctcccaggaccccagacacaagatcacaaagaggggacagaatgtaactttcaggtgtgatccaatttctgaacacaaccgcctttattggtaccgacagaccctggggcagggcccagagtttctgacttacttccagaatgaagctcaactagaaaaatcaaggctgctcagtgatcggttctctgcagagaggcctaagggatctttctccaccttggagatccagcgcacagagcagggggactcggccatgtatctctgtgccagcagccccctagcgggggtcaggtacgagcagtacttcgggccgggcaccaggctcacggtcaca

SEQ ID NO: 213 - DNA, 406 bp, Homo sapiens
  source 1..406: mol_type = other DNA
atgtcactttctagcctgctgaaggtggtcacagcttcactgtggctaggacctggcattgcccagaagataactcaaacccaaccaggaatgttcgtgcaggaaaaggaggctgtgactctggactgcacatatgacaccagtgatccaagttatggtctattctggtacaagcagcccagcagtggggaaatgatttttcttatttatcaggggtcttatgaccagcaaaatgcaacagaaggtcgctactcattgaatttccagaaggcaagaaaatccgccaaccttgtcatctccgcttcacaactgggggactcagcaatgtacttctgtgcaatgagagataggaacaccggtaaccagttctattttgggacagggacaagtttgacggtcattccaa

SEQ ID NO: 214 - DNA, 393 bp, Homo sapiens
  source 1..393: mol_type = other DNA
atgggcttcaggctcctctgctgtgtggccttttgtctcctgggagcaggcccagtggattctggagtcacacaaaccccaaagcacctgatcacagcaactggacagcgagtgacgctgagatgctcccctaggtctggagacctctctgtgtactggtaccaacagagcctggaccagggcctccagttcctcattcagtattataatggagaagagagagcaaaaggaaacattcttgaacgattctccgcacaacagttccctgacttgcactctgaactaaacctgagctctctggagctgggggactcagctttgtatttctgtgccagcagcgtagaggtttacaatgagcagttcttcgggccagggacacggctcaccgtgcta

SEQ ID NO: 215 - protein, 133 aa, Homo sapiens
MRVRLISAVVLCFLGTGLVDMKVTQMPRYLIKRMGENVLLECGQDMSHETMYWYRQDPGLGLQLIYISYDVDSNSEGDIPKGYRVSRKKREHFSLILDSAKTNQTSVYFCASSPRQTNTEVFFGKGTRLTVVE

SEQ ID NO: 216 - protein, 132 aa, Homo sapiens
MKTVTGPLFLCFWLQLNCVSRGEQVEQRPPHLSVREGDSAFIICTYTDSATAYFYWYKQEPGAGLQLLMSVFSNVDRKEEQGLTVLLNKKDKRLSLNLTAAHPGDSAVYFCAVGNSNNRIFFGDGTQLVVKP

SEQ ID NO: 217 - protein, 115 aa, Homo sapiens
MNTKITQSPRYLILGRANKSLECEQHLGHNAMYWYKQSAEKPPELMFLYNLKQLIRNETVPSRFIPECPDSSKLLLHISAVDPEDSAVYFCASSQLGSSAETLYFGSGTRLTVLE

SEQ ID NO: 218 - protein, 132 aa, Homo sapiens
MRPVTCSVLVLLLMLRRSNGDSVTQTEGLVTVTEGLPVKLNCTYQTTYLTIAFFWYVQYLNEAPQVLLKSSTDNKRTEHQGFHATLHKSSSSFHLQKSSAQLSDSALYYCALSDYSNNRLTLGKGTQVVVLP

SEQ ID NO: 219 - protein, 132 aa, Homo sapiens
MGSRLFLVLSLLCTKHMEAAVTQSPRNKVTVTGGNVTLSCRQTNSHNYMYWYRQDTGHGLRLIHYSYGAGNLQIGDVPDGYKATRTTQEDFFLLLELASPSQTSLYFCASSDLGGYNSPLYFAAGTRLTVTE

SEQ ID NO: 220 - DNA, 343 bp, Homo sapiens
  source 1..343: mol_type = other DNA
atgaacactaaaattactcagtcaccaagatatctaatcctgggaagagcaaataagtctttggaatgtgagcaacatctgggacataatgctatgtactggtataaacagagcgctgagaagccgccagagctcatgtttctctacaatcttaaacagttgattcgaaatgagacggtgcccagtcgttttatacctgaatgcccagacagctccaagctacttttacatatatctgccgtggatccagaagactcagctgtctatttttgtgccagcagccaactggggtctagtgcagaaacgctgtattttggctcaggaaccagactgactgttctcg

SEQ ID NO: 221 - DNA, 397 bp, Homo sapiens
  source 1..397: mol_type = other DNA
atgcgtcctgtcacctgctcagttctcgtgctcctcctaatgctcagaaggagcaatggagactccgtgacccagacagaaggcctggtcactgtcaccgaggggttgcctgtgaagctgaactgcacctatcagactacttatttaactattgcctttttctggtatgtgcaatatctcaacgaagcccctcaggtactcctgaagagctccacagacaacaagaggaccgagcaccaagggttccacgccactctccataagagcagcagctccttccatctgcagaagtcctcagcgcagctgtcagactctgccctgtactactgtgctctgagtgactacagcaacaacagacttactttggggaagggaacccaggtggtggtgttaccaa

SEQ ID NO: 222 - DNA, 394 bp, Homo sapiens
  source 1..394: mol_type = other DNA
atgggctccaggctctttctggtcttgagcctcctgtgtacaaaacacatggaggctgcagtcacccaaagccctagaaacaaggtgacagtaacaggaggaaacgtgacattgagctgtcgccagactaatagccacaactacatgtactggtatcggcaggacactgggcatgggctgaggctgatccattactcatatggtgctggcaaccttcaaataggagatgtccctgatgggtacaaggccaccagaacaacgcaagaagacttcttcctcctgctggaattggcttctccctctcagacatctttgtacttctgtgccagcagtgatctggggggctataattcgcccctctactttgcggcaggcacccggctcactgtgacag

SEQ ID NO: 223 - DNA, 397 bp, Homo sapiens
  source 1..397: mol_type = other DNA
atgcgtcctgacacctgctcagttcttgtgctcctcttaatgctcagaaggaacaatggagactctgtgacccagacagaaggcctggtcactctcaccgaggggttgcctgtgatgctgaactgcacctatcagagtacttactcacctttccttttctggtatgtgcaacatctcaacgaagcccctaagctacttttgaagagcttcacagacaacaagaggcccgagcaccaagggttccacgccactctccataagagcagcagctccttccatctgcagaagtcctcagcgcagctgtcagactctgccctgtactactgtgctttgagtgatcggtcgggaaatgagaaaataacttttggggctggaaccaaactcaccattaaaccca

SEQ ID NO: 224 - DNA, 397 bp, Homo sapiens
  source 1..397: mol_type = other DNA
atgagagttaggctcatctctgctgtggtgctgtgtttcctaggaacaggccttgtggacatgaaagtaacccagatgccaagatacctgatcaaaagaatgggagagaatgttttgctggaatgtggacaggacatgagccatgaaacaatgtactggtatcgacaagaccctggtctggggctacagctgatttatatctcatacgatgttgatagtaacagcgaaggagacatccctaaaggatacagggtctcacggaagaagcgggagcatttctccctgattctggattctgctaaaacaaaccagacatctgtgtacttctgtgctagcagtccaagacaaacaaacacagaagtcttctttggtaaaggaaccagactcacagttgtag